European Patent Specification EP 3 532 096 B1, published February 22, 2023. Title: PREFUSION HPIV F IMMUNOGENS AND THEIR USE. Applicant: The United States of America as Represented by the Secretary, Depratment of Health and Human Services. The sequence listing filed with the application follows.

SEQUENCE LISTING (95 sequences)

SEQ ID NO: 1 - protein, 555 aa, human parainfluenza virus 1
MQKSEILFLIYSSLLLSSSLCQIPVDKLSNVGVIINEGKLLKIAGSYESRYIVLSLVPSIDLEDGCGTTQIIQYKNLLNRLLIPLKDALDLQESLITITNDTTVTNDNPQSRFFGAVIGTIALGVATAAQITAGIALAEAREARKDIALIKDSIIKTHNSVELIQRGIGEQIIALKTLQDFVNNEIRPAIGELRCETTALKLGIKLTQHYSELATAFSSNLGTIGEKSLTLQALSSLYSANITEILSTIKKDKSDIYDIIYTEQVKGTVIDVDLEKYMVTLLVKIPILSEIPGVLIYRASSISYNIEGEEWHVAIPNYIINKASSLGGADVTNCIESRLAYICPRDPTQLIPDNQQKCILGDVSKCPVTKVINNLVPKFAFINGGVVANCIASTCTCGTNRIPVNQDRSRGVTFLTYTNCGLIGINGIELYANKRGRDTTWGNQIIKVGPAVSIRPVDISLNLASATNFLEESKIELMKAKAIISAVGGWHNTESTQIIIIIIVCILIIIICGILYYLYRVRRLLVMINSTHNSPVNTYTLESRMRNPYIGNNSN

SEQ ID NO: 2 - protein, 580 aa, human parainfluenza virus 1
MQSSEVLLLVYSSLLLSSSLCQIPVDKLSNVGVIINEGKLLKIAGSYESRYIVLSLVPSIDLQDGCGTTQIIQYKNLLNRLLIPLKDALDLQESLITITNDTTVTNDNPQTRFFGAVIGTIALGVATAAQITAGIALAEAREARKDIALIKDSIVKTHNSVEFIQRGIGEQIIALKTLQDFVNDEIRPAIGELRCETTALKLGIKLTQHYSELATAFSSNLGTIGEKSLTLQALSSLYSANITEILSTIKKDKSDIYDIIYTEQVKGTVIDVDLEKYMVTLLVKIPILSEIPGVLIYRASSISYNIEGEEWHVAIPNYIINKASSLGGADVTNCIESKLAYICPRDPTQLIPDNQQKCILGDVSKCPVTKVINNLVPKFAFINGGVVANCIASTCTCGTNRIPVNQDRSKGVTFLTYTNCGLIGINGIELYANKRGRDTTWGNQIIKVGPAVSIRPVDISLNLASATNFLEESKTELMKARAIISAVGGWHNKESTQIIIIIIVCVLIIIICSILYYLYRVRRLLIMINSTNNSPINAYTLESRMKNPYMGNHSNKIRSSILHTYNNQIYPQLLSDVVRK

SEQ ID NO: 3 - protein, 555 aa, human parainfluenza virus 1
MQSSEILILVYSSLLLSSSLCQIPVDKLSNVGVIINEGKLLKIAGSYESRYIVLSLVPSIDLQDGCGTTQIIQYKNLLNRLLIPLKDALDLQESLITITNDTTVTNDNPQTRFFGAVIGTIALGVATAAQITAGIALAEAREARKDIALIKDSIVKTHNSVEFIQRGIGEQIIALKTLQDFVNDEIPPAIGELRCETTAMKLGIKLTQHYSELATAFSSNLGTIGEKSLTLQALSSLYSANITEILSTIKKDKSDIYDIIYTEQVKGTVIDVDLEKYMVTLLVKIPILSEIPGVLIYRASSISYNIEGEEWHVAIPNYIISKASSLGGADVTNCIESKLAYICPRDPTQLIPDNQQKCILGDVSKCPVTKVINNLVPKFAFINGGVVANCIASTCTCGTNRIPVNQDRSKGVTFLTYTNCGLIGINGIELYGNKRGRDTTWGNQIIKEGPAVSIRPVDISLNLASATNFLEESKTELMKARAIISAVGGWHNTESTQIIIIIIVCILIIIICGILYYLYRVRRLLVMINSTNNSPINAYTLESRMRNPYMGNHSN

SEQ ID NO: 4 - protein, 488 aa, Artificial Sequence
  Recombinant parainfluenza virus F sequence
QIPVDKLSNVGVIINEGKLLKIAGSYESRYIVLSLVPSIDLQDGCGTTQIIQYKNLLNRLLIPLKDALDLQESLITITNDTTVTNDNPQTRGSGAVIGTIALGVATAAQITAGIALAEAREARKDIALIKDSIVKTHNSVEFIQRGIGEQIIALKTLQDFVNDEIRPAIGELRCETTALKLGIKLTQHYSELATAFSSNLGTIGEKSLTLQALSSLYSANITEILSTIKKDKSDIYDIIYTEQVKGTVIDVDLEKYMVTLLVKIPILSEIPGVLIYRASSISYNIEGEEWHVAIPNYIINKASSLGGADVTNCIESKLAYICPRDPTQLIPDNQQKCILGDVSKCPVTKVINNLVPKFAFINGGVVANCIASTCTCGTNRIPVNQDRSKGVTFLTYTNCGLIGINGIELYANKRGRDTTWGNQIIKVGPAVSIRPVDISLNLASITNFLEEIKTELMKIEDKIEEILSKIYHIENEIARIKKLIGEAP

SEQ ID NO: 5 - protein, 551 aa, human parainfluenza virus 2
MHHLHPMIVCIFVMYTGIVGSDAIAGDQLLNIGVIQSKIRSLMYYTDGGASFIVVKLLPNLPPSNGTCNITSLDAYNVTLFKLLTPLIENLSKISTVTDTKTRQKRFAGVVVGLAALGVATAAQITAAVAIVKANANAAAINNLASSIQSTNKAVSDVIDASRTIATAVQAIQDHINGAIVNGITSASCRAHDALIGSILNLYLTELTTIFHNQITNPALTPLSIQALRILLGSTLPIVIESKLNTNLNTAELLSSGLLTGQIISISPMYMQMLIQINVPTFIMQPGAKVIDLIAISANHKLQEVVVQVPNRILEYANELQNYPANDCVVTPNSVCCRYNEGSPIPESQYQCLRGNLNSCTFTPIIGNFLKRFAFANGVLYANCKSLLCRCADPPHVVSQDDTQGISIIDIKRCSEMMLDTFSFRITSTFNATYVTDFSMINANIVHLSPLDLSNQINSINKSLKSAEDWIADSNFFANQARTAKTLYSLSAIALILSVITLVVVGLLIAYIIKLVSQIHQFRSLAATTMFHRENPAFFSKNNHGNIYGIS

SEQ ID NO: 6 - protein, 551 aa, human parainfluenza virus 2
MHHLHPMIVCIFVMYTGIVGSDAIAGDQLLNIGVIQSKIRSLMYYTDGGASFIVVKLLPNLPPSNGTCNITSLDAYNVTLFKLLTPLIENLSKISTVTDTKTRQKRFAGVVVGLAALGVATAAQITAAVAIVKANANAAAINNLASSIQSTNKAVSDVIDASRTIATAVQAIQDRINGAIVNGITSASCRAHDALIGSILNLYLTELTTIFHNQITNPALTPLSIQALRILLGSTLPIVIESKLNTNFNTAELLSSGLLTGQIISISPMYMQMLIQINVPTFIMQPGAKVIDLIAISANHKLQEVVVQVPNRILEYANELQNYPANDCVVTPNSVFCRYNEGSPIPESQYQCLRGNLNSCTFTPIIGNFLKRFAFANGVLYANCKSLLCRCADPPHVVSQDDTQGISIIDIKRCSEMMLDTFSFRITSTFNATYVTDFSMINANIVHLSPLDLSNQINSINKSLKSAEDWIADSNFFANQARTAKTLYSLSAIALILSVITLVVVGLLIAYIIKLVSQIHQFRSLAATTMFHRENPAFFSKNNHGNIYGIS

SEQ ID NO: 7 - protein, 496 aa, Artificial Sequence
  Recombinant parainfluenza virus F sequence
DAIAGDQLLNIGVIQSKIRSLMYYTDGGASFIVVKLLPNLPPSNGTCNITSLDAYNVTLFKLLTPLIENLSKISTVTDTGGGSGGGSGVVVGLAALGVATAAQITAAVAIVKANANAAAINNLASSIQSTNKAVSDVIDASRTIATAVQAIQDRINGAIVNGITSASCRAHDALIGSILNLYLTELTTIFHNQITNPALTPLSIQALRILLGSTLPIVIESKLNTNFNTAELLSSGLLTGQIISISPMYMQMLIQINVPTFIMQPGAKVIDLIAISANHKLQEVVVQVPNRILEYANELQNYPANDCVVTPNSVFCRYNEGSPIPESQYQCLRGNLNSCTFTPIIGNFLKRFAFANGVLYANCKSLLCRCADPPHVVSQDDTQGISIIDIKRCSEMMLDTFSFRITSTFNATYVTDFSMINANIVHLSPLDLSNQINSINKSLKSAEDWIADSNFFANQARTAMKQIEDKIEEILSKIYHIENEIARIKKLIGEAP

SEQ ID NO: 8 - protein, 539 aa, Artificial Sequence
  Recombinant parainfluenza virus F sequence
MPTSILLIITTMIMASFCQIDITKLQHVGVLVNSPKGMKISQNFETRYLILSLIPKIEDSNSCGDQQIKQYKRLLDRLIIPLYDGLRLQKDVIVSNQESNENTDPRTKRFFGGVIGTIALGVATSAQITAAVALVEAKQARSDIEKLKEAIRDTNKAVQSVQSSIGNLIVAIKSVQDYVNKEIVPSIARLGCEAAGLQLGIALTQHYSELTNIFGDNIGSLQEKGIKLQGIASLYRTNITEIFTTSTVDKYDIYDLLFTESIKVRVIDVDLNDYSITLQVRLPLLTRLLNTQIYRVDSISYNIQNREWYIPLPSHIMTKGAFLGGADVKECIEAFSSYICPSDPGFVLNHEMESCLSGNISQCPRTVVKSDIVPRYAFVNGGVVANCITTTCTCNGIGNRINQPPDQGVKIITHKECNTIGINGMLFNTNKEGTLAFYTPNDITLNNSVALDPIDISIELNKAKSDLEESKEWIRRSNQKLDSIGNWHQSSTTIIIVLIMIIILFIINVTIIIIAVKYYRIQKRNRVDQNDKPYVLTNK

SEQ ID NO: 9 - protein, 539 aa, human parainfluenza virus 3
MLISILSIITTMIMASHCQIDITKLQHVGVLVNSPKGMKISQNFETRYLILSLIPKIEDSNSCGDQQIKQYKRLLDRLIIPLYDGLKLQKDVIVTNQESNENTDPRTERFFGGVIGTIALGVATSAQITAAVALVEAKQAKSDIEKLKEAIRDTNKAVQSVQSSVGNLIVAIKSVQDYVNKEIVPSIARLGCEAAGLQLGIALTQHYSELTNIFGDNIGSLQEKGIKLQGIASLYRTNITEIFTTSTVDKYDIYDLLFTESIKVRVIDVDLNDYSITLQVRLPLLTRLLNTQIYKVDSISYNIQNREWYIPLPSHIMTKGAFLGGADVKECIEAFSSYICPSDPGFVLNHEMESCLSGNISQCPRTTVTSDIVPRYAFVNGGVVANCITTTCTCNGIGNRINQPPDQGVKIITHKECNTIGINGMLFNTNKEGTLAFYTPDDITLNNSVALDPIDISIELNKAKSDLEESKEWIRRSNQKLDSIGSWHQSSTTIIIILIMMIILFIINITIITIAIKYYRIQKRNRVDQNDKPYVLTNK

SEQ ID NO: 10 - protein, 495 aa, Artificial Sequence
  Recombinant parainfluenza virus F sequence
QIDITKLQHVGVLVNSPKGMKISQNFETRYLILSLIPKIEDSNSCGDQQIKQYKRLLDRLIIPLYDGLKLQKDVIVTNQESNENTDPRTERFFGGVIGTIALGVATSAQITAAVALVEAKQAKSDILKLKEAIRDTNKAVQSVQSSVGNLIVAIKSVQDYVNKEIVPSIARLGCEAAGLQLGIALTQHYSELTNIFGDNIGSLQEKGIKLQGIASLYRTNITEIFTTSTVDKYDIYDLLFTESIKVRVIDVDLNDYSITLQVRLPLLTRLLNTQIYKVDSISYNIQNREWYIPLPSHIMTKGAFLGGADVKECIEAFSSYICPSDPGFVLNHEMESCLSGNISQCPRTTVTSDIVPRYAFVNGGVVANCITTTCTCNGIGNRINQPPDQGVKIITHKECNTIGINGMLFNTNKEGTLAFYTPDDITLNNSVALDPIDISIELNKAKSDLEESKEWIRRSNQKLSAIEDKIEEILSKIYHIENEIARIKKLIGEAP

SEQ ID NO: 11 - protein, 495 aa, Artificial Sequence
  Recombinant parainfluenza virus F sequence
QIDITKLQHVGVLVNSPKGMKISQNFETRYLILSLIPKIEDSNSCGDQQIKQYKRLLDRLIIPLYDGLKLQKDVIVTNQESNENTDPRTERFFGGVIGTIALGVATSAQITAAVALVEAKQAKSDIEKLKEAIRDTNKAVQSVQSSVGNLIIAIKSVQDYVNKEIVPSIARLGCEAAGLQLGIALTQHYSELTNIFGDNIGSLQEKGIKLQGIASLYRTNITEIFTTSTVDKYDIYDLLFTESIKVRVIDVDLNDYSITLQVRLPLLTRLLNTQIYKVDSISYNIQNREWYIPLPSHIMTKGAFLGGADVKECIEAFSSYICPSDPGFVLNHEMESCLSGNISQCPRTTVTSDIVPRYAFVNGGVVANCITTTCTCNGIGNRINQPPDQGVKIITHKECNTIGINGMLFNTNKEGTLAFYTPDDITLNNSVALDPIDISIELNKAKSDLEESKEWIRRSNQKLSAIEDKIEEILSKIYHIENEIARIKKLIGEAP

SEQ ID NO: 12 - protein, 495 aa, Artificial Sequence
  Recombinant parainfluenza virus F sequence
QIDITKLQHVGVLVNSPKGMKISQNFETRYLILSLIPKIEDSNSCGDQQIKQYKRLLDRLIIPLYDGLKLQKDVIVTNQESNENTDPRTERFFGGVIGTIALGVATSAQITAAVALVEAKQAKSDIEKLKEAIRDTNKAVQSVQSSVGNLIVAIKSIQDYVNKEIVPSIARLGCEAAGLQLGIALTQHYSELTNIFGDNIGSLQEKGIKLQGIASLYRTNITEIFTTSTVDKYDIYDLLFTESIKVRVIDVDLNDYSITLQVRLPLLTRLLNTQIYKVDSISYNIQNREWYIPLPSHIMTKGAFLGGADVKECIEAFSSYICPSDPGFVLNHEMESCLSGNISQCPRTTVTSDIVPRYAFVNGGVVANCITTTCTCNGIGNRINQPPDQGVKIITHKECNTIGINGMLFNTNKEGTLAFYTPDDITLNNSVALDPIDISIELNKAKSDLEESKEWIRRSNQKLSAIEDKIEEILSKIYHIENEIARIKKLIGEAP

SEQ ID NO: 13 - protein, 495 aa, Artificial Sequence
  Recombinant parainfluenza virus F sequence
QIDITKLQHVGVLVNSPKGMKISQNFETRYLILSLIPKIEDSNSCGDQQIKQYKRLLDRLIIPLYDGLKLQKDVIVTNQESNENTDPRTERFFGGVIGTIALGVATSAQITAAVALVEAKQAKSDIEKLKEAIRDTNKAVQSVQSSVGNLIVAIKSVQDWVNKEIVPSIARLGCEAAGLQLGIALTQHYSELTNIFGDNIGSLQEKGIKLQGIASLYRTNITEIFTTSTVDKYDIYDLLFTESIKVRVIDVDLNDYSITLQVRLPLLTRLLNTQIYKVDSISYNIQNREWYIPLPSHIMTKGAFLGGADVKECIEAFSSYICPSDPGFVLNHEMESCLSGNISQCPRTTVTSDIVPRYAFVNGGVVANCITTTCTCNGIGNRINQPPDQGVKIITHKECNTIGINGMLFNTNKEGTLAFYTPDDITLNNSVALDPIDISIELNKAKSDLEESKEWIRRSNQKLSAIEDKIEEILSKIYHIENEIARIKKLIGEAP

SEQ ID NO: 14 - protein, 495 aa, Artificial Sequence
  Recombinant parainfluenza virus F sequence
QIDITKLQHVGVLVNSPKGMKISQNFETRYLILSLIPKIEDSNSCGDQQIKQYKRLLDRLIIPLYDGLKLQKDVIVTNQESNENTDPRTERFFGGVIGTIALGVATSAQITAAVALVEAKQAKSDIEKLKEAIRDTNKAVQSVQSSVGNLIVAIKSVQDYVNKEIVPSIARLGCPAAGLQLGIALTQHYSELTNIFGDNIGSLQEKGIKLQGIASLYRTNITEIFTTSTVDKYDIYDLLFTESIKVRVIDVDLNDYSITLQVRLPLLTRLLNTQIYKVDSISYNIQNREWYIPLPSHIMTKGAFLGGADVKECIEAFSSYICPSDPGFVLNHEMESCLSGNISQCPRTTVTSDIVPRYAFVNGGVVANCITTTCTCNGIGNRINQPPDQGVKIITHKECNTIGINGMLFNTNKEGTLAFYTPDDITLNNSVALDPIDISIELNKAKSDLEESKEWIRRSNQKLSAIEDKIEEILSKIYHIENEIARIKKLIGEAP

SEQ ID NO: 15 - protein, 495 aa, Artificial Sequence
  Recombinant parainfluenza virus F sequence
QIDITKLQHVGVLVNSPKGMKISQNFETRYLILSLIPKIEDSNSCGDQQIKQYKRLLDRLIIPLYDGLKLQKDVIVTNQESNENTDPRTERFFGGVIGTIALGVATSAQITAAVALVEAKQAKSDIEKLKEAIRDTNKAVQSVQSSVGNLIVAIKSVQDYVNKEIVPSIARLGCEAAGLQLGIALTQHYSELTNIFGDNIGSLQEKGIKLQGIASLYRTNITEIFTTSTVDKYDIYDLLFTESIKVRVIDVDLNDYSITLQVRLPLLTRLLNTQIYKVDSISYNIQNREWYIPLPSHIMTKGAFLGGADVKECIEAFSSYICPSDPGFVLNHEMESCLSGNISQCPRTTVTSDIVPRYAFVNGGVVANCITTTCTCNGIGNRINQPPDQGVKIITHKECNTIGINGMLFNTNKEGTLAFYTPDDITLNNSVALDPIDISIELNKVKSDLEESKEWIRRSNQKLSAIEDKIEEILSKIYHIENEIARIKKLIGEAP

SEQ ID NO: 16 - protein, 495 aa, Artificial Sequence
  Recombinant parainfluenza virus F sequence
QIDITKLQHVGVLVNSPKGMKISQNFETRYLILSLIPKIEDSNSCGDQQIKQYKRLLDRLIIPLYDGLKLQKDVIVTNQESNENTDPRTERFFGGVIGTIALGVATSAQITAAVALVEAKQAKSDIEKLKEAIRDTNKAVQSVQSSVGNLIVAIKSVQDYVNKEIVPSIARLGCEAAGLQLGIALTQHYSELTNIFGDNIGSLQEKGIKLQGIASLYRTNITEIFTTSTVDKYDIYDLLFTESIKVRVIDVDLNDYSITLQVRLPLLTRLLNTQIYKVDSISYNIQNREWYIPLPSHIMTKGAFLGGADVKECIEAFSSYICPSDPGFVLNHEMESCLSGNISQCPRTTVTSDIVPRYAFVNGGVVANCITTTCTCNGIGNRINQPPDQGVKIITHKECNTIGINGMLFNTNKEGTLAFYTPDDITLNNSVALDPIDISIELNKAKSDLEELKEWIRRSNQKLSAIEDKIEEILSKIYHIENEIARIKKLIGEAP

SEQ ID NO: 17 - protein, 495 aa, Artificial Sequence
  Recombinant parainfluenza virus F sequence
QIDITKLQHVGVLVNSPKGMKISQNFETRYLILSLIPKIEDSNSCGDQQIKQYKRLLDRLIIPLYDGLKLQKDVIVTNQESNENTDPRTERFFGGVIGTIALGVATSAQITAAVALVEAKQAKSDIEKLKEAIRDTNKAVQSVQSSVGNLIVAIKSVQDYVNKEIVPSIARLGCEAAGLQLGIALTQHYSELTNIFGDNIGSLQEKGIKLQGIASLYRTNITEIFTTSTVDKYDIYDLLFTESIKVRVIDVDLNDYSITLQVRLPLLTRLLNTQIYKVDSISYNIQNREWYIPLPSHIMTKGAFLGGADVKECIEAFSSYICPSDPGFVLNHEMESCLSGNISQCPRTTVTSDIVPRYAFVNGGVVANCITTTCTCNGIGNRINQPPDQGVKIITHKECNTIGINGMLFNTNKEGTLAFYTPDDITLNNSVALDPIDISIELNKAKSDLEEVKEWIRRSNQKLSAIEDKIEEILSKIYHIENEIARIKKLIGEAP

SEQ ID NO: 18 - protein, 495 aa, Artificial Sequence
  Recombinant parainfluenza virus F sequence
QIDITKLQHVGVLVNSPKGMKISQNFETRYLILSLIPKIEDSNSCGDQQIKQYKRLLDRLIIPLYDGLKLQKDVIVTNQESNENTDPRTERFFGGVIGTIALGVATSAQITAAVALVEAKQAKSDIEKLKEAIRDTNKAVQSVQSSVGNLIVAIKSVQDYVNKEIVPSIARLGCEAAGLQLGIALTQHYSELTNIFGDNIGSLQEKGIKLQGIASLYRTNITEIFTTSTVDKYDIYDLLFTESIKVRVIDVDLNDYSITLQVRLPLLTRLLNTQIYKVDSISYNIQNREWYIPLPSHIMTKGAFLGGADVKECIEAFSSYICPSDPGFVLNHEMESCLSGNISQCPRTTVTSDIVPRYAFVNGGVVANCITTTCTCNGIGNRINQPPDQGVKIITHKECNTIGINGMLFNTNKEGTLAFYTPDDITLNNSVALDPIDISIELNKAKSDLEESKEWYRRSNQKLSAIEDKIEEILSKIYHIENEIARIKKLIGEAP

SEQ ID NO: 19 - protein, 495 aa, Artificial Sequence
  Recombinant parainfluenza virus F sequence
QIDITKLQHVGVLVNSPKGMKISQNFETRYLILSLIPKIEDSNSCGDQQIKQYKRLLDRLIIPLYDGLKLQKDVIVTNQESNENTDPRTERFFGGVIGTIALGVATSAQITAAVALVEAKQAKSDIEKLKEAIRDTNKAVQSVQSSVGNLIVAIKSVQDYVNKEIVPSIARLGCEAAGLQLGIALTQHYSELTNIFGDNIGSLQEKGIKLQGIASLYRTNITEIFTTSTVDKYDIYDLLFTESIKVRVIDVDLNDYSITLQVRLPLLTRLLNTQIYKVDSISYNIQNREWYIPLPSHIMTKGAFLGGADVKECIEAFSSYICPSDPGFVLNHEMESCLSGNISQCPRTTVTSDIVPRYAFVNGGVVANCITTTCTCNGIGNRINQPPDQGVKIITHKECNTIGINGMLFNTNKEGTLAFYTPDDITLNNSVALDPIDISIELNKAKSDLEESKEWIRRVNQKLSAIEDKIEEILSKIYHIENEIARIKKLIGEAP

SEQ ID NO: 20 - protein, 495 aa, Artificial Sequence
  Recombinant parainfluenza virus F sequence
QIDITKLQHVGVLVNSPKGMKISQNFETRYLILSLIPKIEDSNSCGDQQIKQYKRLLDRLIIPLYDGLKLQKDVIVTNQESNENTDPRTERFFGGVIGTIALGVATSAQITAAVALVEAKQAKSDIEKLKEAIRDTNKAVQSVQSSVGNLIVAIKSVQDYVNKEIVPSIARLGCEAAGLQLGIALTQHYSELTNIFGDNIGSLQEKGIKLQGIASLYRTNITEIFTTSTVDKYDIYDLLFTESIKVRVIDVDLNDYSITLQVRLPLLTRLLNTQIYKVDSISYNIQNREWYIPLPSHIMTKGAFLGGADVKECIEAFSSYICPSDPGFVLNHEMESCLSGNISQCPRTTVTSDIVPRYAFVNGGVVANCITTTCTCNGIGNRINQPPDQGVKIITHKECNTIGINGMLFNTNKEGTLAFYTPDDITLNNSVALDPIDISIELNKVKSDLEESKEWYRRSNQKLSAIEDKIEEILSKIYHIENEIARIKKLIGEAP

SEQ ID NO: 21 - protein, 495 aa, Artificial Sequence
  Recombinant parainfluenza virus F sequence
QIDITKLQHVGVLVNSPKGMKISQNFETRYLILSLIPKIEDSNSCGDQQIKQYKRLLDRLIIPLYDGLKLQKDVIVTNQESNENTDPRTERFFGGVIGTIALGVATSAQITAAVALVEAKQAKSDIEKLKEAIRDTNKAVQSVQSSVGNLIVAIKSVQDWVNKEIVPSIARLGCEAAGLQLGIALTQHYSELTNIFGDNIGSLQEKGIKLQGIASLYRTNITEIFTTSTVDKYDIYDLLFTESIKVRVIDVDLNDYSITLQVRLPLLTRLLNTQIYKVDSISYNIQNREWYIPLPSHIMTKGAFLGGADVKECIEAFSSYICPSDPGFVLNHEMESCLSGNISQCPRTTVTSDIVPRYAFVNGGVVANCITTTCTCNGIGNRINQPPDQGVKIITHKECNTIGINGMLFNTNKEGTLAFYTPDDITLNNSVALDPIDISIELNKVKSDLEESKEWYRRSNQKLSAIEDKIEEILSKIYHIENEIARIKKLIGEAP

SEQ ID NO: 22 - protein, 495 aa, Artificial Sequence
  Recombinant parainfluenza virus F sequence
QIDITKLQHVGVLVNSPKGMKISQNFETRYLILSLIPKIEDSNSCGDQQIKQYKRLLDRLIIPLYDGLKLQKDVIVTNQESNENTDPRTERFFGGVIGTIALGVATSAQITAAVALVEAKQAKSDIEKLKEAIRDTNKAVQSVQSSVGNLIVACKSVQDYVNKEIVPSIARLGCEAAGLQLGIALTQHYSELTNIFGDNIGSLQEKGIKLQGIASLYRTCITEIFTTSTVDKYDIYDLLFTESIKVRVIDVDLNDYSITLQVRLPLLTRLLNTQIYKVDSISYNIQNREWYIPLPSHIMTKGAFLGGADVKECIEAFSSYICPSDPGFVLNHEMESCLSGNISQCPRTTVTSDIVPRYAFVNGGVVANCITTTCTCNGIGNRINQPPDQGVKIITHKECNTIGINGMLFNTNKEGTLAFYTPDDITLNNSVALDPIDISIELNKAKSDLEESKEWIRRSNQKLSAIEDKIEEILSKIYHIENEIARIKKLIGEAP

SEQ ID NO: 23 - protein, 495 aa, Artificial Sequence
  Recombinant parainfluenza virus F sequence
QIDITKLQHVGVLVNSPKGMKISQNFETRYLILSLIPKIEDSNSCGDQQIKQYKRLLDRLIIPLYDGLKLQKDVIVTNQESNENTDPRTERFFGGVIGTIALGVATSAQITAAVALVEAKQAKSDIEKLKEAIRDTNKAVQSVQSSVGNLILACKSVQDYVNKEIVPSFARLGCEAAGLQLGIALTQHYSELTNIFGDNIGSLQEKGIKLQGIASLYRTCITEIFTTSTVDKYDIYDLLFTESIKVRVIDVDLNDYSITLQVRLPLLTRLLNTQIYKVDSISYNIQNREWYIPLPSHIMTKGAFLGGADVKECIEAFSSYICPSDPGFVLNHEMESCLSGNISQCPRTTVTSDIVPRYAFVNGGVVANCITTTCTCNGIGNRINQPPDQGVKIITHKECNTIGINGMLFNTNKEGTLAFYTPDDITLNNSVALDPIDISIELNKAKSDLEESKEWIRRSNQKLSAIEDKIEEILSKIYHIENEIARIKKLIGEAP

SEQ ID NO: 24 - protein, 495 aa, Artificial Sequence; identical to SEQ ID NO: 13
  Recombinant parainfluenza virus F sequence

SEQ ID NO: 25 - protein, 495 aa, Artificial Sequence
  Recombinant parainfluenza virus F sequence
QIDITKLQHVGVLVNSPKGMKISQNFETRYLILSLIPKIEDSNSCGDQQIKQYKRLLDRLIIPLYDGLKLQKDVIVTNQESNENTDPRTERFFGGVIGTIALGVATSAQITAAVALVEAKQAKSDIEKLKEAIRDTNKAVQSVQSSVGNLIVACKSVQDYVNKEIVPSIARLGCEAAGLQLGIALTQHYSELTNIFGDNIGSLQEKGIKLQGIASLYRTCITEIFTTSTVDKYDIYDLLFTESIKVRVIDVDLNDYSITLQVRLPLLTRLLNTQIYKVDSISYNIQNREWYIPLPSHIMTKGAFLGGADVKECIEAFSSYICPSDPGFVLNHEMESCLSGNISQCPRTTVTSDIVPRYAFVNGGVVANCITTTCTCNGIGNRINQPPDQGVKIITHKECNTIGINGMLFNTNKEGTLAFYTPDDITLNNSVALDPIDISIELNKAKSDLEESKEWYRRSNQKLSAIEDKIEEILSKIYHIENEIARIKKLIGEAP

SEQ ID NO: 26 - protein, 495 aa, Artificial Sequence
  Recombinant parainfluenza virus F sequence
QIDITKLQHVGVLVNSPKGMKISQNFETRYLILSLIPKIEDSNSCGDQQIKQYKRLLDRLIIPLYDGLKLQKDVIVTNQESNENTDPRTERFFGGVIGTIALGVATSAQITAAVALVEAKQAKSDIEKLKEAIRDTNKAVQSVQSSVGNLIVACKSVQDYVNKEIVPSIARLGCEAAGLQLGIALTQHYSELTNIFGDNIGSLQEKGIKLQGIASLYRTCITEIFTTSTVDKYDIYDLLFTESIKVRVIDVDLNDYSITLQVRLPLLTRLLNTQIYKVDSISYNIQNREWYIPLPSHIMTKGAFLGGADVKECIEAFSSYICPSDPGFVLNHEMESCLSGNISQCPRTTVTSDIVPRYAFVNGGVVANCITTTCTCNGIGNRINQPPDQGVKIITHKECNTIGINGMLFNTNKEGTLAFYTPDDITLNNSVALDPIDISIELNKVKSDLEESKEWYRRSNQKLSAIEDKIEEILSKIYHIENEIARIKKLIGEAP

SEQ ID NO: 27 - protein, 544 aa, human parainfluenza virus 4
MGVKGSSLIMIGLLISPITNLDITHLMNLGTVPTAIRSLVYYTYTKPSYLTVDLIPNLKNLDQNCNYSSLNYYNKTALSLIQPIADNINRLTKPIASSEVQSRFFGAVIGTIALGVATAAQVTAAIGLAKAQENAKLILTLKKAATETNEAVRDLANSNKIVVKMISAIQNQINTIIQPAIDQINCQIKDLQVANILNLYLTEITTVFHNQLTNPALESISIQALKSLLGSTLPEVLSKLDLNNISAASVMASGLIKGQIIAVDIPTMTLVLMVQIPSISPLRQAKIIDLTSITIHTNSQEVQAVVPARFLEIGSEILGFDGSVCQITKDTIFCPYNDAYVLPIQQKRCLQGQTRDCVFTPVAGTFPRRFLTTYGTIVANCRDLVCSCLRPPQIIYQPDENPVTIIDKDLCTTLTLDSITIEIQKSINSTFRREVVLESTQVRSLTPLDLSTDLNQYNQLLKSAEDHIQRSTDYLNSINPSIVNNNAIIILIILCILLILTVTICIIWLKYLTNEVKNVARNQRLNRDADLFHRIPSQIPVPRQ

SEQ ID NO: 28 - protein, 544 aa, human parainfluenza virus 4
MGVKGSSLIMIGLLISPITNLDITHLMNLGTVPTAIRSLVYYTYTKPSYLTVDLIPNLKNLDQNCNYSSLNYYNKTALSLIQPIADNINRLTKPITSSEVQSRFFGAVIGTIALGVATAAQVTAAIGLAKAQENAKLILTLKKAATETNEAVRDLANSNKIVVKMISAIQNQINTIIQPAIDQINCQIKDLQVANILNLYLTEITTVFHNQLTNPALESISIQALKSLLGSTLPEVLSKLDLNNISAASVMASGLIKGQIIAVDIPTMTLVLMVQIPSISPLRQAKIIDLTSITIHTNSQEVQAVVPARVLEIGSEILGFDGSVCQITKDTVFCPYNDAYVLPIQQKRCLQGQTRDCVFTPVAGTFPRRFLTTYGTIVANCRDLVCSCLRPPQIIYQPDENPVTIIDKDLCTTLTLDSITIEIQKSINSTFRREVVLESTQVRSLTPLDLSTDLNQYNQLLKSAEDHIQRSTDYLNSINPSIVNNNAIIILIILCILLILTVTICIIWLKYLTNEVKNVARNQRLNRDADLFHRIPSQIPVPRQ

SEQ ID NO: 29 - protein, 487 aa, Artificial Sequence
  Recombinant parainfluenza virus F sequence
LDITHLMNLGTVPTAIRSLVYYTYTKPSYLTVDLIPNLKNLDQNCNYSSLNYYNKTALSLIQPIADNINRLTKPITSGGGSGGGSGAVIGTIALGVATAAQVTAAIGLAKAQENAKLILTLKKAATETNEAVRDLANSNKIVVKMISAIQNQINTIIQPAIDQINCQIKDLQVANILNLYLTEITTVFHNQLTNPALESISIQALKSLLGSTLPEVLSKLDLNNISAASVMASGLIKGQIIAVDIPTMTLVLMVQIPSISPLRQAKIIDLTSITIHTNSQEVQAVVPARVLEIGSEILGFDGSVCQITKDTVFCPYNDAYVLPIQQKRCLQGQTRDCVFTPVAGTFPRRFLTTYGTIVANCRDLVCSCLRPPQIIYQPDENPVTIIDKDLCTTLTLDSITIEIQKSINSTFRREVVLESTQVRSLTPLDLSTDLNQFNQLLKSAEDHIQRVTDYLNSIEDKIEEILSKIYHIENEIARIKKLIGEAP

SEQ ID NO: 30 - protein, 487 aa, Artificial Sequence
  Recombinant parainfluenza virus F sequence
LDITHLMNLGTVPTAIRSLVYYTYTKPSYLTVDLIPNLKNLDQNCNYSSLNYYNKTALSLIQPIADNINRLTKPITSGGGSGGGSGAVIGTIALGVATAAQVTAAIGLAKAQENAKLILTLKKAATETNEAVRDLANSNKIVVKMCSAIQNQINTIIQPAIDQINCQIKDLQVANILNLYLTEITTVFHNQLTNPALESISIQALKSLLGSCLPEVLSKLDLNNISAASVMASGLIKGQIIAVDIPTMTLVLMVQIPSISPLRQAKIIDLTSITIHTNSQEVQAVVPARVLEIGSEILGFDGSVCQITKDTVFCPYNDAYVLPIQQKRCLQGQTRDCVFTPVAGTFPRRFLTTYGTIVANCRDLVCSCLRPPQIIYQPDENPVTIIDKDLCTTLTLDSITIEIQKSINSTFRREVVLESTQVRSLTPLDLSTDLNQFNQLLKSAEDHIQRVTDYLNSIEDKIEEILSKIYHIENEIARIKKLIGEAP

SEQ ID NO: 31 - protein, 33 aa, Artificial Sequence
  GCN4 trimerization domain
MKQVEDKIEEILSKIYHIENEIARIKKLIGEAP

SEQ ID NO: 32 - protein, 8 aa, Artificial Sequence
  Peptide linker
GGGSGGGS

SEQ ID NO: 33 - protein, 8 aa, Artificial Sequence
  parainfluenza virus F peptide
KTRQKRFA

SEQ ID NO: 34 - protein, 8 aa, Artificial Sequence
  parainfluenza virus F peptide
SEVQSRFF

SEQ ID NO: 35 - protein, 173 aa, Artificial Sequence
  Self-assembling protein nanoparticle sequence
ESQVRQQFSKDIEKLLNEQVNKEMQSSNLYMSMSSWCYTHSLDGAGLFLFDHAAEEYEHAKKLIIFLNENNVPVQLTSISAPEHKFEGLTQIFQKAYEHEQHISESINNIVDHAIKSKDHATFNFLQWYVAEQHEEEVLFKDILDKIELIGNENHGLYLADQYVKGIAKSRKS

SEQ ID NO: 36 - protein, 154 aa, Artificial Sequence
  Self-assembling protein nanoparticle sequence
MQIYEGKLTAEGLRFGIVASRFNHALVDRLVEGAIDAIVRHGGREEDITLVRVPGSWEIPVAAGELARKEDIDAVIAIGVLIRGATPHFDYIASEVSKGLADLSLELRKPITFGVITADTLEQAIERAGTKHGNKGWEAALSAIEMANLFKSLR

SEQ ID NO: 37 - protein, 265 aa, Artificial Sequence [sequence omitted]

SEQ ID NO: 38 - protein, 265 aa, Artificial Sequence [sequence omitted]

SEQ ID NO: 39 - protein, 495 aa, Artificial Sequence
  Recombinant parainfluenza virus F sequence
QIDITKLQHVGVLVNSPKGMKISQNFETRYLILSLIPKIEDSNSCGDQQIKQYKRLLDRLIIPLYDGLKLQKDVIVTNQESNENTDPRTERFFGGVIGTIALGVATSAQITAAVALVEAKQAKSDIEKLKEAIRDTNKAVQSVQSSVGNLICAIKSVQDYVNKEIVPSIARLGCEAAGLQLGIALTQHYSELTNIFGDNIGSLQEKGIKLQGIASLYRTNITECFTTSTVDKYDIYDLLFTESIKVRVIDVDLNDYSITLQVRLPLLTRLLNTQIYKVDSISYNIQNREWYIPLPSHIMTKGAFLGGADVKECIEAFSSYICPSDPGFVLNHEMESCLSGNISQCPRTTVTSDIVPRYAFVNGGVVANCITTTCTCNGIGNRINQPPDQGVKIITHKECNTIGINGMLFNTNKEGTLAFYTPDDITLNNSVALDPIDISIELNKVKSDLEESKEWYRRSNQKLSAIEDKIEEILSKIYHIENEIARIKKLIGEAP

SEQ ID NO: 40 - protein, 495 aa, Artificial Sequence
  Recombinant parainfluenza virus F sequence
QIDITKLQHVGVLVNSPKGMKISQNFETRYLILSLIPKIEDSNSCGDQQIKQYKRLLDRLIIPLYDGLKLQKDVIVTNQESNENTDPRTERFFGGVIGTIALGVATSAQITAAVALVEAKQAKSDIEKLKEAIRDTNKAVQSVQSSVGNLIVAIKSVQDYVNKEIVPSIARLGCEAAGLQLGIALTQHYSELTNCFGDNIGSLQEKGIKLQCIASLYRTNITEIFTTSTVDKYDIYDLLFTESIKVRVIDVDLNDYSITLQVRLPLLTRLLNTQIYKVDSISYNIQNREWYIPLPSHIMTKGAFLGGADVKECIEAFSSYICPSDPGFVLNHEMESCLSGNISQCPRTTVTSDIVPRYAFVNGGVVANCITTTCTCNGIGNRINQPPDQGVKIITHKECNTIGINGMLFNTNKEGTLAFYTPDDITLNNSVALDPIDISIELNKVKSDLEESKEWYRRSNQKLSAIEDKIEEILSKIYHIENEIARIKKLIGEAP

SEQ ID NO: 41 - protein, 495 aa, Artificial Sequence
  Recombinant parainfluenza virus F sequence
QIDITKLQHVGVLVNSPKGMKISQNFETRYLILSLIPKIEDSNSCGDQQIKQYKRLLDRLIIPLYDCLKLQKDVIVTNQESNENTDPRTERFFGGVIGTIALGVATSAQITAAVALVEAKQAKSDIEKLKEAIRDTNKAVQSVQSSVGNLIVAIKSVQDYVNKEIVPSIARLGCEAAGLQLGIALTQHYSELTNIFGDNIGSLCEKGIKLQGIASLYRTNITEIFTTSTVDKYDIYDLLFTESIKVRVIDVDLNDYSITLQVRLPLLTRLLNTQIYKVDSISYNIQNREWYIPLPSHIMTKGAFLGGADVKECIEAFSSYICPSDPGFVLNHEMESCLSGNISQCPRTTVTSDIVPRYAFVNGGVVANCITTTCTCNGIGNRINQPPDQGVKIITHKECNTIGINGMLFNTNKEGTLAFYTPDDITLNNSVALDPIDISIELNKVKSDLEESKEWYRRSNQKLSAIEDKIEEILSKIYHIENEIARIKKLIGEAP

SEQ ID NO: 42 - protein, 495 aa, Artificial Sequence
  Recombinant parainfluenza virus F sequence
QIDITKLQHVGVLVNSPKGMKISQNFETRYLILSLIPKIEDSNSCGDQQIKQYKRLLDRLIIPLYDGLKLQKDVIVTNQESNENTDPRTERFFGGVIGTIALGVATSAQITAAVALVEAKQAKSDIEKLKEAIRDTNKAVQSVQSSVGNLIVAIKSVQDYVNKEIVPSIARLGCEAAGLQLGIALTQHYSELTNIFGCNIGSCQEKGIKLQGIASLYRTNITEIFTTSTVDKYDIYDLLFTESIKVRVIDVDLNDYSITLQVRLPLLTRLLNTQIYKVDSISYNIQNREWYIPLPSHIMTKGAFLGGADVKECIEAFSSYICPSDPGFVLNHEMESCLSGNISQCPRTTVTSDIVPRYAFVNGGVVANCITTTCTCNGIGNRINQPPDQGVKIITHKECNTIGINGMLFNTNKEGTLAFYTPDDITLNNSVALDPIDISIELNKVKSDLEESKEWYRRSNQKLSAIEDKIEEILSKIYHIENEIARIKKLIGEAP

SEQ ID NO: 43 - protein, 495 aa, Artificial Sequence
  Recombinant parainfluenza virus F sequence
QIDITKLQHVGVLVNSPKGMKISQNFETRYLILSLIPKIEDSNSCGDQQIKQYKRLLDRLIIPLYDGLKLQKDVIVTNQESNENTDPRTERFFGGVIGTIALGVATSAQITAAVALVEAKQAKSDIEKLKEAIRDTNKAVQSVCSSVGNCIVAIKSVQDYVNKEIVPSIARLGCEAAGLQLGIALTQHYSELTNIFGDNIGSLQEKGIKLQGIASLYRTNITEIFTTSTVDKYDIYDLLFTESIKVRVIDVDLNDYSITLQVRLPLLTRLLNTQIYKVDSISYNIQNREWYIPLPSHIMTKGAFLGGADVKECIEAFSSYICPSDPGFVLNHEMESCLSGNISQCPRTTVTSDIVPRYAFVNGGVVANCITTTCTCNGIGNRINQPPDQGVKIITHKECNTIGINGMLFNTNKEGTLAFYTPDDITLNNSVALDPIDISIELNKVKSDLEESKEWYRRSNQKLSAIEDKIEEILSKIYHIENEIARIKKLIGEAP

SEQ ID NO: 44 - protein, 495 aa, Artificial Sequence
  Recombinant parainfluenza virus F sequence
QIDITKLQHVGVLVNSPKGMKISQNFETRYLILSLIPKIEDSNSCGDQQIKQYKRLLDRLIIPLYDGLKLQKDVIVTNQESNENTDPRTERFFGGVIGTIALGVATSAQITAAVALVEAKQAKSDIEKLKEAIRDTNKAVQSVCSSVGNCICAIKSVQDYVNKEIVPSIARLGCEAAGLQLGIALTQHYSELTNIFGDNIGSLQEKGIKLQGIASLYRTNITECFTTSTVDKYDIYDLLFTESIKVRVIDVDLNDYSITLQVRLPLLTRLLNTQIYKVDSISYNIQNREWYIPLPSHIMTKGAFLGGADVKECIEAFSSYICPSDPGFVLNHEMESCLSGNISQCPRTTVTSDIVPRYAFVNGGVVANCITTTCTCNGIGNRINQPPDQGVKIITHKECNTIGINGMLFNTNKEGTLAFYTPDDITLNNSVALDPIDISIELNKVKSDLEESKEWYRRSNQKLSAIEDKIEEILSKIYHIENEIARIKKLIGEAP

SEQ ID NO: 45 - protein, 495 aa, Artificial Sequence
  Recombinant parainfluenza virus F sequence
QIDITKLQHVGVLVNSPKGMKISQNFETRYLILSLIPKIEDSNSCGDQQIKQYKRLLDRLIIPLYDGLKLQKDVIVTNQESNENTDPRTERFFGGVIGTIALGVATSAQITAAVALVEAKQAKSDIEKLKEAIRDTNKAVQSVCSSVGNCIVAIKSVQDYVNKEIVPSIARLGCEAAGLQLGIALTQHYSELTNCFGDNIGSLQEKGIKLQCIASLYRTNITEIFTTSTVDKYDIYDLLFTESIKVRVIDVDLNDYSITLQVRLPLLTRLLNTQIYKVDSISYNIQNREWYIPLPSHIMTKGAFLGGADVKECIEAFSSYICPSDPGFVLNHEMESCLSGNISQCPRTTVTSDIVPRYAFVNGGVVANCITTTCTCNGIGNRINQPPDQGVKIITHKECNTIGINGMLFNTNKEGTLAFYTPDDITLNNSVALDPIDISIELNKVKSDLEESKEWYRRSNQKLSAIEDKIEEILSKIYHIENEIARIKKLIGEAP

SEQ ID NO: 46 - protein, 495 aa, Artificial Sequence
  Recombinant parainfluenza virus F sequence
QIDITKLQHVGVLVNSPKGMKISQNFETRYLILSLIPKIEDSNSCGDQQIKQYKRLLDRLIIPLYDGLKLQKDVIVTNQESNENTDPRTERFFGGVIGTIALGVATSAQITAAVALVEAKQAKSDIEKLKEAIRDTNKAVQSVCSSVGNCIVAIKSVQDYVNKEIVPSIARLGCEAAGLQLGIALTQHYSELTNIFGCNIGSCQEKGIKLQGIASLYRTNITEIFTTSTVDKYDIYDLLFTESIKVRVIDVDLNDYSITLQVRLPLLTRLLNTQIYKVDSISYNIQNREWYIPLPSHIMTKGAFLGGADVKECIEAFSSYICPSDPGFVLNHEMESCLSGNISQCPRTTVTSDIVPRYAFVNGGVVANCITTTCTCNGIGNRINQPPDQGVKIITHKECNTIGINGMLFNTNKEGTLAFYTPDDITLNNSVALDPIDISIELNKVKSDLEESKEWYRRSNQKLSAIEDKIEEILSKIYHIENEIARIKKLIGEAP

SEQ ID NO: 47 - protein, 495 aa, Artificial Sequence
  Recombinant parainfluenza virus F sequence
QIDITKLQHVGVLVNSPKGMKISQNFETRYLILSLIPKIEDSNSCGDQQIKQYKRLLDRLIIPLYDCLKLQKDVIVTNQESNENTDPRTERFFGGVIGTIALGVATSAQITAAVALVEAKQAKSDIEKLKEAIRDTNKAVQSVCSSVGNCIVAIKSVQDYVNKEIVPSIARLGCEAAGLQLGIALTQHYSELTNIFGDNIGSLCEKGIKLQGIASLYRTNITEIFTTSTVDKYDIYDLLFTESIKVRVIDVDLNDYSITLQVRLPLLTRLLNTQIYKVDSISYNIQNREWYIPLPSHIMTKGAFLGGADVKECIEAFSSYICPSDPGFVLNHEMESCLSGNISQCPRTTVTSDIVPRYAFVNGGVVANCITTTCTCNGIGNRINQPPDQGVKIITHKECNTIGINGMLFNTNKEGTLAFYTPDDITLNNSVALDPIDISIELNKVKSDLEESKEWYRRSNQKLSAIEDKIEEILSKIYHIENEIARIKKLIGEAP

SEQ ID NO: 48 - protein, 495 aa, Artificial Sequence
  Recombinant parainfluenza virus F sequence
QIDITKLQHVGVLVNSPKGMKISQNFETRYLILSLIPKIEDSNSCGDQQIKQYKRLLDRLIIPLYDGLKLQKDVIVTNQESNENTDPRTERFFGGVIGTIALGVATSAQITAAVALVEAKQAKSDIEKLKEAIRDTNKAVQSVQSSVGNLICAIKSVQDYVNKEIVPSIARLGCEAAGLQLGIALTQHYSELTNCFGDNIGSLQEKGIKLQCIASLYRTNITECFTTSTVDKYDIYDLLFTESIKVRVIDVDLNDYSITLQVRLPLLTRLLNTQIYKVDSISYNIQNREWYIPLPSHIMTKGAFLGGADVKECIEAFSSYICPSDPGFVLNHEMESCLSGNISQCPRTTVTSDIVPRYAFVNGGVVANCITTTCTCNGIGNRINQPPDQGVKIITHKECNTIGINGMLFNTNKEGTLAFYTPDDITLNNSVALDPIDISIELNKVKSDLEESKEWYRRSNQKLSAIEDKIEEILSKIYHIENEIARIKKLIGEAP

SEQ ID NO: 49 - protein, 495 aa, Artificial Sequence
  Recombinant parainfluenza virus F sequence
QIDITKLQHVGVLVNSPKGMKISQNFETRYLILSLIPKIEDSNSCGDQQIKQYKRLLDRLIIPLYDGLKLQKDVIVTNQESNENTDPRTERFFGGVIGTIALGVATSAQITAAVALVEAKQAKSDIEKLKEAIRDTNKAVQSVQSSVGNLIVAIKSVQDYVNKEIVPSIARLGCEAAGLQLGIALTQHYSELTNCFGCNIGSCQEKGIKLQCIASLYRTNITEIFTTSTVDKYDIYDLLFTESIKVRVIDVDLNDYSITLQVRLPLLTRLLNTQIYKVDSISYNIQNREWYIPLPSHIMTKGAFLGGADVKECIEAFSSYICPSDPGFVLNHEMESCLSGNISQCPRTTVTSDIVPRYAFVNGGVVANCITTTCTCNGIGNRINQPPDQGVKIITHKECNTIGINGMLFNTNKEGTLAFYTPDDITLNNSVALDPIDISIELNKVKSDLEESKEWYRRSNQKLSAIEDKIEEILSKIYHIENEIARIKKLIGEAP

SEQ ID NO: 50 - protein, 495 aa, Artificial Sequence
  Recombinant parainfluenza virus F sequence
QIDITKLQHVGVLVNSPKGMKISQNFETRYLILSLIPKIEDSNSCGDQQIKQYKRLLDRLIIPLYDCLKLQKDVIVTNQESNENTDPRTERFFGGVIGTIALGVATSAQITAAVALVEAKQAKSDIEKLKEAIRDTNKAVQSVQSSVGNLIVAIKSVQDYVNKEIVPSIARLGCEAAGLQLGIALTQHYSELTNCFGDNIGSLCEKGIKLQCIASLYRTNITEIFTTSTVDKYDIYDLLFTESIKVRVIDVDLNDYSITLQVRLPLLTRLLNTQIYKVDSISYNIQNREWYIPLPSHIMTKGAFLGGADVKECIEAFSSYICPSDPGFVLNHEMESCLSGNISQCPRTTVTSDIVPRYAFVNGGVVANCITTTCTCNGIGNRINQPPDQGVKIITHKECNTIGINGMLFNTNKEGTLAFYTPDDITLNNSVALDPIDISIELNKVKSDLEESKEWYRRSNQKLSAIEDKIEEILSKIYHIENEIARIKKLIGEAP

SEQ ID NO: 51 - protein, 521 aa, Artificial Sequence
  Recombinant parainfluenza virus F sequence
QIDITKLQHVGVLVNSPKGMKISQNFETRYLILSLIPKIEDSNSCGDQQIKQYKRLLDRLIIPLYDGLKLQKDVIVTNQESNENTDPRTERFFGGVIGTIALGVATSAQITAAVALVEAKQAKSDIEKLKEAIRDTNKAVQSVQSSVGNLIVAIKSVQDYVNKEIVPSIARLGCEAAGLQLGIALTQHYSELTNIFGDNIGSLQEKGIKLQGIASLYRTNITEIFTTSTVDKYDIYDLLFTESIKVRVIDVDLNDYSITLQVRLPLLTRLLNTQIYKVDSISYNIQNREWYIPLPSHIMTKGAFLGGADVKECIEAFSSYICPSDPGFVLNHEMESCLSGNISQCPRTTVTSDIVPRYAFVNGGVVANCITTTCTCNGIGNRINQPPDQGVKIITHKECNTIGINGMLFNTNKEGTLAFYTPDDITLNNSVALDPIDISIELNKVKSDLEESKEWYRRSNQKLDSIGSWHQSSTTIIIILIMMIILFIINITIITIAIKYYRIQKRNRVDQNDKPYVLTNK

SEQ ID NO: 52 - protein, 521 aa, Artificial Sequence
  Recombinant parainfluenza virus F sequence
QIDITKLQHVGVLVNSPKGMKISQNFETRYLILSLIPKIEDSNSCGDQQIKQYKRLLDRLIIPLYDGLKLQKDVIVTNQESNENTDPRTERFFGGVIGTIALGVATSAQITAAVALVEAKQAKSDIEKLKEAIRDTNKAVQSVQSSVGNLIVACKSVQDYVNKEIVPSIARLGCEAAGLQLGIALTQHYSELTNIFGDNIGSLQEKGIKLQGIASLYRTCITEIFTTSTVDKYDIYDLLFTESIKVRVIDVDLNDYSITLQVRLPLLTRLLNTQIYKVDSISYNIQNREWYIPLPSHIMTKGAFLGGADVKECIEAFSSYICPSDPGFVLNHEMESCLSGNISQCPRTTVTSDIVPRYAFVNGGVVANCITTTCTCNGIGNRINQPPDQGVKIITHKECNTIGINGMLFNTNKEGTLAFYTPDDITLNNSVALDPIDISIELNKAKSDLEESKEWIRRSNQKLDSIGSWHQSSTTIIIILIMMIILFIINITIITIAIKYYRIQKRNRVDQNDKPYVLTNK

SEQ ID NO: 53 - protein, 521 aa, Artificial Sequence
  Recombinant parainfluenza virus F sequence
QIDITKLQHVGVLVNSPKGMKISQNFETRYLILSLIPKIEDSNSCGDQQIKQYKRLLDRLIIPLYDGLKLQKDVIVTNQESNENTDPRTERFFGGVIGTIALGVATSAQITAAVALVEAKQAKSDIEKLKEAIRDTNKAVQSVQSSVGNLIVACKSVQDYVNKEIVPSIARLGCEAAGLQLGIALTQHYSELTNIFGDNIGSLQEKGIKLQGIASLYRTCITEIFTTSTVDKYDIYDLLFTESIKVRVIDVDLNDYSITLQVRLPLLTRLLNTQIYKVDSISYNIQNREWYIPLPSHIMTKGAFLGGADVKECIEAFSSYICPSDPGFVLNHEMESCLSGNISQCPRTTVTSDIVPRYAFVNGGVVANCITTTCTCNGIGNRINQPPDQGVKIITHKECNTIGINGMLFNTNKEGTLAFYTPDDITLNNSVALDPIDISIELNKVKSDLEESKEWYRRSNQKLDSIGSWHQSSTTIIIILIMMIILFIINITIITIAIKYYRIQKRNRVDQNDKPYVLTNK

SEQ ID NO: 54 - protein, 521 aa, Artificial Sequence
  Recombinant parainfluenza virus F sequence
QIDITKLQHVGVLVNSPKGMKISQNFETRYLILSLIPKIEDSNSCGDQQIKQYKRLLDRLIIPLYDGLKLQKDVIVTNQESNENTDPRTERFFGGVIGTIALGVATSAQITAAVALVEAKQAKSDIEKLKEAIRDTNKAVQSVQSSVGNLICAIKSVQDYVNKEIVPSIARLGCEAAGLQLGIALTQHYSELTNIFGDNIGSLQEKGIKLQGIASLYRTNITECFTTSTVDKYDIYDLLFTESIKVRVIDVDLNDYSITLQVRLPLLTRLLNTQIYKVDSISYNIQNREWYIPLPSHIMTKGAFLGGADVKECIEAFSSYICPSDPGFVLNHEMESCLSGNISQCPRTTVTSDIVPRYAFVNGGVVANCITTTCTCNGIGNRINQPPDQGVKIITHKECNTIGINGMLFNTNKEGTLAFYTPDDITLNNSVALDPIDISIELNKVKSDLEESKEWYRRSNQKLDSIGSWHQSSTTIIIILIMMIILFIINITIITIAIKYYRIQKRNRVDQNDKPYVLTNK

SEQ ID NO: 55 - protein, 521 aa, Artificial Sequence
  Recombinant parainfluenza virus F sequence
QIDITKLQHVGVLVNSPKGMKISQNFETRYLILSLIPKIEDSNSCGDQQIKQYKRLLDRLIIPLYDGLKLQKDVIVTNQESNENTDPRTERFFGGVIGTIALGVATSAQITAAVALVEAKQAKSDIEKLKEAIRDTNKAVQSVQSSVGNLIVAIKSVQDYVNKEIVPSIARLGCEAAGLQLGIALTQHYSELTNCFGDNIGSLQEKGIKLQCIASLYRTNITEIFTTSTVDKYDIYDLLFTESIKVRVIDVDLNDYSITLQVRLPLLTRLLNTQIYKVDSISYNIQNREWYIPLPSHIMTKGAFLGGADVKECIEAFSSYICPSDPGFVLNHEMESCLSGNISQCPRTTVTSDIVPRYAFVNGGVVANCITTTCTCNGIGNRINQPPDQGVKIITHKECNTIGINGMLFNTNKEGTLAFYTPDDITLNNSVALDPIDISIELNKVKSDLEESKEWYRRSNQKLDSIGSWHQSSTTIIIILIMMIILFIINITIITIAIKYYRIQKRNRVDQNDKPYVLTNK

SEQ ID NO: 56 - protein, 521 aa, Artificial Sequence
  Recombinant parainfluenza virus F sequence
QIDITKLQHVGVLVNSPKGMKISQNFETRYLILSLIPKIEDSNSCGDQQIKQYKRLLDRLIIPLYDCLKLQKDVIVTNQESNENTDPRTERFFGGVIGTIALGVATSAQITAAVALVEAKQAKSDIEKLKEAIRDTNKAVQSVQSSVGNLIVAIKSVQDYVNKEIVPSIARLGCEAAGLQLGIALTQHYSELTNIFGDNIGSLCEKGIKLQGIASLYRTNITEIFTTSTVDKYDIYDLLFTESIKVRVIDVDLNDYSITLQVRLPLLTRLLNTQIYKVDSISYNIQNREWYIPLPSHIMTKGAFLGGADVKECIEAFSSYICPSDPGFVLNHEMESCLSGNISQCPRTTVTSDIVPRYAFVNGGVVANCITTTCTCNGIGNRINQPPDQGVKIITHKECNTIGINGMLFNTNKEGTLAFYTPDDITLNNSVALDPIDISIELNKVKSDLEESKEWYRRSNQKLDSIGSWHQSSTTIIIILIMMIILFIINITIITIAIKYYRIQKRNRVDQNDKPYVLTNK

SEQ ID NO: 57 - protein, 521 aa, Artificial Sequence
  Recombinant parainfluenza virus F sequence
QIDITKLQHVGVLVNSPKGMKISQNFETRYLILSLIPKIEDSNSCGDQQIKQYKRLLDRLIIPLYDGLKLQKDVIVTNQESNENTDPRTERFFGGVIGTIALGVATSAQITAAVALVEAKQAKSDIEKLKEAIRDTNKAVQSVQSSVGNLIVAIKSVQDYVNKEIVPSIARLGCEAAGLQLGIALTQHYSELTNIFGCNIGSCQEKGIKLQGIASLYRTNITEIFTTSTVDKYDIYDLLFTESIKVRVIDVDLNDYSITLQVRLPLLTRLLNTQIYKVDSISYNIQNREWYIPLPSHIMTKGAFLGGADVKECIEAFSSYICPSDPGFVLNHEMESCLSGNISQCPRTTVTSDIVPRYAFVNGGVVANCITTTCTCNGIGNRINQPPDQGVKIITHKECNTIGINGMLFNTNKEGTLAFYTPDDITLNNSVALDPIDISIELNKVKSDLEESKEWYRRSNQKLDSIGSWHQSSTTIIIILIMMIILFIINITIITIAIKYYRIQKRNRVDQNDKPYVLTNK

SEQ ID NO: 58 - protein, 521 aa, Artificial Sequence
  Recombinant parainfluenza virus F sequence
QIDITKLQHVGVLVNSPKGMKISQNFETRYLILSLIPKIEDSNSCGDQQIKQYKRLLDRLIIPLYDGLKLQKDVIVTNQESNENTDPRTERFFGGVIGTIALGVATSAQITAAVALVEAKQAKSDIEKLKEAIRDTNKAVQSVCSSVGNCIVAIKSVQDYVNKEIVPSIARLGCEAAGLQLGIALTQHYSELTNIFGDNIGSLQEKGIKLQGIASLYRTNITEIFTTSTVDKYDIYDLLFTESIKVRVIDVDLNDYSITLQVRLPLLTRLLNTQIYKVDSISYNIQNREWYIPLPSHIMTKGAFLGGADVKECIEAFSSYICPSDPGFVLNHEMESCLSGNISQCPRTTVTSDIVPRYAFVNGGVVANCITTTCTCNGIGNRINQPPDQGVKIITHKECNTIGINGMLFNTNKEGTLAFYTPDDITLNNSVALDPIDISIELNKVKSDLEESKEWYRRSNQKLDSIGSWHQSSTTIIIILIMMIILFIINITIITIAIKYYRIQKRNRVDQNDKPYVLTNK

SEQ ID NO: 59 - protein, 521 aa, Artificial Sequence
  Recombinant parainfluenza virus F sequence
QIDITKLQHVGVLVNSPKGMKISQNFETRYLILSLIPKIEDSNSCGDQQIKQYKRLLDRLIIPLYDGLKLQKDVIVTNQESNENTDPRTERFFGGVIGTIALGVATSAQITAAVALVEAKQAKSDIEKLKEAIRDTNKAVQSVCSSVGNCICAIKSVQDYVNKEIVPSIARLGCEAAGLQLGIALTQHYSELTNIFGDNIGSLQEKGIKLQGIASLYRTNITECFTTSTVDKYDIYDLLFTESIKVRVIDVDLNDYSITLQVRLPLLTRLLNTQIYKVDSISYNIQNREWYIPLPSHIMTKGAFLGGADVKECIEAFSSYICPSDPGFVLNHEMESCLSGNISQCPRTTVTSDIVPRYAFVNGGVVANCITTTCTCNGIGNRINQPPDQGVKIITHKECNTIGINGMLFNTNKEGTLAFYTPDDITLNNSVALDPIDISIELNKVKSDLEESKEWYRRSNQKLDSIGSWHQSSTTIIIILIMMIILFIINITIITIAIKYYRIQKRNRVDQNDKPYVLTNK

SEQ ID NO: 60 - protein, 521 aa, Artificial Sequence
  Recombinant parainfluenza virus F sequence
QIDITKLQHVGVLVNSPKGMKISQNFETRYLILSLIPKIEDSNSCGDQQIKQYKRLLDRLIIPLYDGLKLQKDVIVTNQESNENTDPRTERFFGGVIGTIALGVATSAQITAAVALVEAKQAKSDIEKLKEAIRDTNKAVQSVCSSVGNCIVAIKSVQDYVNKEIVPSIARLGCEAAGLQLGIALTQHYSELTNCFGDNIGSLQEKGIKLQCIASLYRTNITEIFTTSTVDKYDIYDLLFTESIKVRVIDVDLNDYSITLQVRLPLLTRLLNTQIYKVDSISYNIQNREWYIPLPSHIMTKGAFLGGADVKECIEAFSSYICPSDPGFVLNHEMESCLSGNISQCPRTTVTSDIVPRYAFVNGGVVANCITTTCTCNGIGNRINQPPDQGVKIITHKECNTIGINGMLFNTNKEGTLAFYTPDDITLNNSVALDPIDISIELNKVKSDLEESKEWYRRSNQKLDSIGSWHQSSTTIIIILIMMIILFIINITIITIAIKYYRIQKRNRVDQNDKPYVLTNK

SEQ ID NO: 61 - protein, 521 aa, Artificial Sequence
  Recombinant parainfluenza virus F sequence
QIDITKLQHVGVLVNSPKGMKISQNFETRYLILSLIPKIEDSNSCGDQQIKQYKRLLDRLIIPLYDGLKLQKDVIVTNQESNENTDPRTERFFGGVIGTIALGVATSAQITAAVALVEAKQAKSDIEKLKEAIRDTNKAVQSVCSSVGNCIVAIKSVQDYVNKEIVPSIARLGCEAAGLQLGIALTQHYSELTNIFGCNIGSCQEKGIKLQGIASLYRTNITEIFTTSTVDKYDIYDLLFTESIKVRVIDVDLNDYSITLQVRLPLLTRLLNTQIYKVDSISYNIQNREWYIPLPSHIMTKGAFLGGADVKECIEAFSSYICPSDPGFVLNHEMESCLSGNISQCPRTTVTSDIVPRYAFVNGGVVANCITTTCTCNGIGNRINQPPDQGVKIITHKECNTIGINGMLFNTNKEGTLAFYTPDDITLNNSVALDPIDISIELNKVKSDLEESKEWYRRSNQKLDSIGSWHQSSTTIIIILIMMIILFIINITIITIAIKYYRIQKRNRVDQNDKPYVLTNK

SEQ ID NO: 62 - protein, 521 aa, Artificial Sequence
  Recombinant parainfluenza virus F sequence
QIDITKLQHVGVLVNSPKGMKISQNFETRYLILSLIPKIEDSNSCGDQQIKQYKRLLDRLIIPLYDCLKLQKDVIVTNQESNENTDPRTERFFGGVIGTIALGVATSAQITAAVALVEAKQAKSDIEKLKEAIRDTNKAVQSVCSSVGNCIVAIKSVQDYVNKEIVPSIARLGCEAAGLQLGIALTQHYSELTNIFGDNIGSLCEKGIKLQGIASLYRTNITEIFTTSTVDKYDIYDLLFTESIKVRVIDVDLNDYSITLQVRLPLLTRLLNTQIYKVDSISYNIQNREWYIPLPSHIMTKGAFLGGADVKECIEAFSSYICPSDPGFVLNHEMESCLSGNISQCPRTTVTSDIVPRYAFVNGGVVANCITTTCTCNGIGNRINQPPDQGVKIITHKECNTIGINGMLFNTNKEGTLAFYTPDDITLNNSVALDPIDISIELNKVKSDLEESKEWYRRSNQKLDSIGSWHQSSTTIIIILIMMIILFIINITIITIAIKYYRIQKRNRVDQNDKPYVLTNK

SEQ ID NO: 63 - protein, 521 aa, Artificial Sequence
  Recombinant parainfluenza virus F sequence
QIDITKLQHVGVLVNSPKGMKISQNFETRYLILSLIPKIEDSNSCGDQQIKQYKRLLDRLIIPLYDGLKLQKDVIVTNQESNENTDPRTERFFGGVIGTIALGVATSAQITAAVALVEAKQAKSDIEKLKEAIRDTNKAVQSVQSSVGNLICAIKSVQDYVNKEIVPSIARLGCEAAGLQLGIALTQHYSELTNCFGDNIGSLQEKGIKLQCIASLYRTNITECFTTSTVDKYDIYDLLFTESIKVRVIDVDLNDYSITLQVRLPLLTRLLNTQIYKVDSISYNIQNREWYIPLPSHIMTKGAFLGGADVKECIEAFSSYICPSDPGFVLNHEMESCLSGNISQCPRTTVTSDIVPRYAFVNGGVVANCITTTCTCNGIGNRINQPPDQGVKIITHKECNTIGINGMLFNTNKEGTLAFYTPDDITLNNSVALDPIDISIELNKVKSDLEESKEWYRRSNQKLDSIGSWHQSSTTIIIILIMMIILFIINITIITIAIKYYRIQKRNRVDQNDKPYVLTNK

SEQ ID NO: 64 - protein, 521 aa, Artificial Sequence
  Recombinant parainfluenza virus F sequence
QIDITKLQHVGVLVNSPKGMKISQNFETRYLILSLIPKIEDSNSCGDQQIKQYKRLLDRLIIPLYDGLKLQKDVIVTNQESNENTDPRTERFFGGVIGTIALGVATSAQITAAVALVEAKQAKSDIEKLKEAIRDTNKAVQSVQSSVGNLIVAIKSVQDYVNKEIVPSIARLGCEAAGLQLGIALTQHYSELTNCFGCNIGSCQEKGIKLQCIASLYRTNITEIFTTSTVDKYDIYDLLFTESIKVRVIDVDLNDYSITLQVRLPLLTRLLNTQIYKVDSISYNIQNREWYIPLPSHIMTKGAFLGGADVKECIEAFSSYICPSDPGFVLNHEMESCLSGNISQCPRTTVTSDIVPRYAFVNGGVVANCITTTCTCNGIGNRINQPPDQGVKIITHKECNTIGINGMLFNTNKEGTLAFYTPDDITLNNSVALDPIDISIELNKVKSDLEESKEWYRRSNQKLDSIGSWHQSSTTIIIILIMMIILFIINITIITIAIKYYRIQKRNRVDQNDKPYVLTNK

SEQ ID NO: 65 - protein, 521 aa, Artificial Sequence
  Recombinant parainfluenza virus F sequence
QIDITKLQHVGVLVNSPKGMKISQNFETRYLILSLIPKIEDSNSCGDQQIKQYKRLLDRLIIPLYDCLKLQKDVIVTNQESNENTDPRTERFFGGVIGTIALGVATSAQITAAVALVEAKQAKSDIEKLKEAIRDTNKAVQSVQSSVGNLIVAIKSVQDYVNKEIVPSIARLGCEAAGLQLGIALTQHYSELTNCFGDNIGSLCEKGIKLQCIASLYRTNITEIFTTSTVDKYDIYDLLFTESIKVRVIDVDLNDYSITLQVRLPLLTRLLNTQIYKVDSISYNIQNREWYIPLPSHIMTKGAFLGGADVKECIEAFSSYICPSDPGFVLNHEMESCLSGNISQCPRTTVTSDIVPRYAFVNGGVVANCITTTCTCNGIGNRINQPPDQGVKIITHKECNTIGINGMLFNTNKEGTLAFYTPDDITLNNSVALDPIDISIELNKVKSDLEESKEWYRRSNQKLDSIGSWHQSSTTIIIILIMMIILFIINITIITIAIKYYRIQKRNRVDQNDKPYVLTNK

SEQ ID NO: 66 - protein, 540 aa, bovine parainfluenza virus 3
MIIIVITMILSLTPSSLCQIDITKLQSVGVLVNSPKGIKISQNFETRYLILSLIPKIEDSHSCGNQQIDQYKKLLDRLIIPLYDGLKLQKDVIVVNHESHNNTNLRTKRFFGEIIGTIAIGIATSAQITAAVALVEAKQARSDIDKLKEAIKDTNKAVQSIQSSVGNLIVAVKSVQDYVNNEIVPSITRLGCEAAGLQLGIALTQHYSELTNIFGDNIGTLGEKGVKLQGIASLYRTNITEVFTTSTVDQYDIYDLLFTESIKMRVIDVDLSDYSITLQVRLPLLTKVSNTQIYKVDSISYNIQGKEWYIPLPHHIMTKGAFLGGADIKECIESFSNYICPSDPGFILNHEMENCLSGNITQCPKTIVTSDIVPRYAFVDGGVIANCIPTTCTCNGIDNRINQSPDQGIKIITYKECQIVGINGMLFKTNQEGTLAKYTFDNIKLNNSVALNPIDISLELNKAKSDLEESKRWIEKSNQKLDSIGSWHQSSVTIIIIIVMIVVLLIINAIIIMIMIRYLRDRNRHLNNKDSEPYVLTNRQ

SEQ ID NO: 67 - protein, 540 aa, bovine parainfluenza virus 3
MIITVITVILLLTPSSLCQIDITKLQNVGVLVNSPKGIKISQNFETRYLILSLIPKIDDSHSCGNQQIDQYKKLLDRLIIPLYDGLKLQRDVIVVNHESHNNTNLRTKRFFGEIIGTIAIGIATSAQITAAVALVEAKQARSDIDKLKEAIKDTNKAVQSIQSSVGNLIVAVKSVQDYVNNEIVPSITRLGCEAAGLQLGIALTQHYSELTNIFGDNIGTLREKGVKLQGIASLYRTNITEVFTTSTVDQYDIYDLLFTESIKMRVIDVDLSDYSITLQVRLPLLTKVSNTQIYKVDSISYNIQGKEWYIPLPHHIMTKGAFLGGADIKECIESFSNYICPSDPGFILNHELENCLSGNITQCPKTIVTSDIVPRYAFVDGGVIANCIPTTCTCNGIDNRINQSPDQGIKIITYKECQIVGINGMLFKTNQEGTLAKYTFDDIKLNNSVALNPIDISLELNKAKSELEESKRWIEKSNHKLDSIGSWYQSSATIIIIIVMIVVLLIINAIIIMITIKHLRARNRHPNNKDSEPYVLTNRQ

SEQ ID NO: 68 - protein, 541 aa, caprine parainfluenza virus 3
MIKKIICIFSMPILLSFCQVDIIKLQRVGILVSKPKSIKISQNFETRYLVLNLIPNIENAQSCGDQQIKQYKKLLDRLIIPLYDGLRLQQDIIVVDNNLKNNTNHRAKRFFGEIIGTIALGVATSAQITAAVALVEAKQARSDIERVKNAVRDTNKAVQSIQGSVGNLIVAVKSVQDYVNNEIVPSIKRLGCEAAGLQLGIALTQHYSELTNIFGDNIGTLKEKGIKLQGIASLYHTNITEIFTTSTVDQYDIYDLLFTESIKMRVIDVDLNDYSITLQVRLPLLTKISDAQIYNVDSVSYNIGGTEWYIPLPRNIMTKGAFLGGANLQDCIESFSDYICPSDPGFILNRDIENCLSGNITQCPKTLVISDIVPRYAFVDGGVIANCLSTTCTCNGIDNRINQAPDQGIKIITYKDCQTIGINGMLFKTNQEGTLAAYTPVDITLNNSVNLDPIDLSIELNRARSDLAESKEWIKRSEAKLDSVGSWYQSSTTEIIQIVMIIVLFIINIIVLIVLIKYSRSQNQSMNNHMNEPYILTNKVQ

SEQ ID NO: 69 - protein, 495 aa, Artificial Sequence
  Recombinant parainfluenza virus F sequence
QIDITKLQSVGVLVNSPKGIKISQNFETRYLILSLIPKIEDSHSCGNQQIDQYKKLLDRLIIPLYDGLKLQKDVIVVNHESHNNTNLRTKRFFGEIIGTIAIGIATSAQITAAVALVEAKQARSDIDKLKEAIKDTNKAVQSIQSSVGNLIVACKSVQDYVNNEIVPSITRLGCEAAGLQLGIALTQHYSELTNIFGDNIGTLGEKGVKLQGIASLYRTCITEVFTTSTVDQYDIYDLLFTESIKMRVIDVDLSDYSITLQVRLPLLTKVSNTQIYKVDSISYNIQGKEWYIPLPHHIMTKGAFLGGADIKECIESFSNYICPSDPGFILNHEMENCLSGNITQCPKTIVTSDIVPRYAFVDGGVIANCIPTTCTCNGIDNRINQSPDQGIKIITYKECQIVGINGMLFKTNQEGTLAKYTFDNIKLNNSVALNPIDISLELNKAKSDLEESKRWYEKSNQKLSAIEDKIEEILSKIYHIENEIARIKKLIGEAP

SEQ ID NO: 70 - protein, 495 aa, Artificial Sequence
  Recombinant parainfluenza virus F sequence
QIDITKLQNVGVLVNSPKGIKISQNFETRYLILSLIPKIDDSHSCGNQQIDQYKKLLDRLIIPLYDGLKLQRDVIVVNHESHNNTNLRTKRFFGEIIGTIAIGIATSAQITAAVALVEAKQARSDIDKLKEAIKDTNKAVQSIQSSVGNLIVACKSVQDYVNNEIVPSITRLGCEAAGLQLGIALTQHYSELTNIFGDNIGTLREKGVKLQGIASLYRTCITEVFTTSTVDQYDIYDLLFTESIKMRVIDVDLSDYSITLQVRLPLLTKVSNTQIYKVDSISYNIQGKEWYIPLPHHIMTKGAFLGGADIKECIESFSNYICPSDPGFILNHELENCLSGNITQCPKTIVTSDIVPRYAFVDGGVIANCIPTTCTCNGIDNRINQSPDQGIKIITYKECQIVGINGMLFKTNQEGTLAKYTFDDIKLNNSVALNPIDISLELNKAKSELEESKRWYEKSNHKLSAIEDKIEEILSKIYHIENEIARIKKLIGEAP

SEQ ID NO: 71 - protein, 495 aa, Artificial Sequence
  Recombinant parainfluenza virus F sequence
QVDIIKLQRVGILVSKPKSIKISQNFETRYLVLNLIPNIENAQSCGDQQIKQYKKLLDRLIIPLYDGLRLQQDIIVVDNNLKNNTNHRAKRFFGEIIGTIALGVATSAQITAAVALVEAKQARSDIERVKNAVRDTNKAVQSIQGSVGNLIVACKSVQDYVNNEIVPSIKRLGCEAAGLQLGIALTQHYSELTNIFGDNIGTLKEKGIKLQGIASLYHTCITEIFTTSTVDQYDIYDLLFTESIKMRVIDVDLNDYSITLQVRLPLLTKISDAQIYNVDSVSYNIGGTEWYIPLPRNIMTKGAFLGGANLQDCIESFSDYICPSDPGFILNRDIENCLSGNITQCPKTLVISDIVPRYAFVDGGVIANCLSTTCTCNGIDNRINQAPDQGIKIITYKDCQTIGINGMLFKTNQEGTLAAYTPVDITLNNSVNLDPIDLSIELNRARSDLAESKEWYKRSEAKLSAIEDKIEEILSKIYHIENEIARIKKLIGEAP

SEQ ID NO: 72 - protein, 495 aa, Artificial Sequence
  Recombinant parainfluenza virus F sequence
QIDITKLQSVGVLVNSPKGIKISQNFETRYLILSLIPKIEDSHSCGNQQIDQYKKLLDRLIIPLYDGLKLQKDVIVVNHESHNNTNLRTKRFFGEIIGTIAIGIATSAQITAAVALVEAKQARSDIDKLKEAIKDTNKAVQSIQSSVGNLIVACKSVQDYVNNEIVPSITRLGCEAAGLQLGIALTQHYSELTNIFGDNIGTLGEKGVKLQGIASLYRTCITEVFTTSTVDQYDIYDLLFTESIKMRVIDVDLSDYSITLQVRLPLLTKVSNTQIYKVDSISYNIQGKEWYIPLPHHIMTKGAFLGGADIKECIESFSNYICPSDPGFILNHEMENCLSGNITQCPKTIVTSDIVPRYAFVDGGVIANCIPTTCTCNGIDNRINQSPDQGIKIITYKECQIVGINGMLFKTNQEGTLAKYTFDNIKLNNSVALNPIDISLELNKVKSDLEESKRWIEKSNQKLSAIEDKIEEILSKIYHIENEIARIKKLIGEAP

SEQ ID NO: 73 - protein, 495 aa, Artificial Sequence
  Recombinant parainfluenza virus F sequence
QIDITKLQNVGVLVNSPKGIKISQNFETRYLILSLIPKIDDSHSCGNQQIDQYKKLLDRLIIPLYDGLKLQRDVIVVNHESHNNTNLRTKRFFGEIIGTIAIGIATSAQITAAVALVEAKQARSDIDKLKEAIKDTNKAVQSIQSSVGNLIVACKSVQDYVNNEIVPSITRLGCEAAGLQLGIALTQHYSELTNIFGDNIGTLREKGVKLQGIASLYRTCITEVFTTSTVDQYDIYDLLFTESIKMRVIDVDLSDYSITLQVRLPLLTKVSNTQIYKVDSISYNIQGKEWYIPLPHHIMTKGAFLGGADIKECIESFSNYICPSDPGFILNHELENCLSGNITQCPKTIVTSDIVPRYAFVDGGVIANCIPTTCTCNGIDNRINQSPDQGIKIITYKECQIVGINGMLFKTNQEGTLAKYTFDDIKLNNSVALNPIDISLELNKVKSELEESKRWIEKSNHKLSAIEDKIEEILSKIYHIENEIARIKKLIGEAP

SEQ ID NO: 74 - protein, 495 aa, Artificial Sequence
  Recombinant parainfluenza virus F sequence
QVDIIKLQRVGILVSKPKSIKISQNFETRYLVLNLIPNIENAQSCGDQQIKQYKKLLDRLIIPLYDGLRLQQDIIVVDNNLKNNTNHRAKRFFGEIIGTIALGVATSAQITAAVALVEAKQARSDIERVKNAVRDTNKAVQSIQGSVGNLIVACKSVQDYVNNEIVPSIKRLGCEAAGLQLGIALTQHYSELTNIFGDNIGTLKEKGIKLQGIASLYHTCITEIFTTSTVDQYDIYDLLFTESIKMRVIDVDLNDYSITLQVRLPLLTKISDAQIYNVDSVSYNIGGTEWYIPLPRNIMTKGAFLGGANLQDCIESFSDYICPSDPGFILNRDIENCLSGNITQCPKTLVISDIVPRYAFVDGGVIANCLSTTCTCNGIDNRINQAPDQGIKIITYKDCQTIGINGMLFKTNQEGTLAAYTPVDITLNNSVNLDPIDLSIELNRVRSDLAESKEWIKRSEAKLSAIEDKIEEILSKIYHIENEIARIKKLIGEAP

SEQ ID NO: 75 - protein, 522 aa, Artificial Sequence
  Recombinant parainfluenza virus F sequence
QIDITKLQSVGVLVNSPKGIKISQNFETRYLILSLIPKIEDSHSCGNQQIDQYKKLLDRLIIPLYDGLKLQKDVIVVNHESHNNTNLRTKRFFGEIIGTIAIGIATSAQITAAVALVEAKQARSDIDKLKEAIKDTNKAVQSIQSSVGNLIVACKSVQDYVNNEIVPSITRLGCEAAGLQLGIALTQHYSELTNIFGDNIGTLGEKGVKLQGIASLYRTCITEVFTTSTVDQYDIYDLLFTESIKMRVIDVDLSDYSITLQVRLPLLTKVSNTQIYKVDSISYNIQGKEWYIPLPHHIMTKGAFLGGADIKECIESFSNYICPSDPGFILNHEMENCLSGNITQCPKTIVTSDIVPRYAFVDGGVIANCIPTTCTCNGIDNRINQSPDQGIKIITYKECQIVGINGMLFKTNQEGTLAKYTFDNIKLNNSVALNPIDISLELNKAKSDLEESKRWYEKSNQKLDSIGSWHQSSVTIIIIIVMIVVLLIINAIIIMIMIRYLRDRNRHLNNKDSEPYVLTNRQ

SEQ ID NO: 76 - protein, 522 aa, Artificial Sequence
  Recombinant parainfluenza virus F sequence
QIDITKLQNVGVLVNSPKGIKISQNFETRYLILSLIPKIDDSHSCGNQQIDQYKKLLDRLIIPLYDGLKLQRDVIVVNHESHNNTNLRTKRFFGEIIGTIAIGIATSAQITAAVALVEAKQARSDIDKLKEAIKDTNKAVQSIQSSVGNLIVACKSVQDYVNNEIVPSITRLGCEAAGLQLGIALTQHYSELTNIFGDNIGTLREKGVKLQGIASLYRTCITEVFTTSTVDQYDIYDLLFTESIKMRVIDVDLSDYSITLQVRLPLLTKVSNTQIYKVDSISYNIQGKEWYIPLPHHIMTKGAFLGGADIKECIESFSNYICPSDPGFILNHELENCLSGNITQCPKTIVTSDIVPRYAFVDGGVIANCIPTTCTCNGIDNRINQSPDQGIKIITYKECQIVGINGMLFKTNQEGTLAKYTFDDIKLNNSVALNPIDISLELNKAKSELEESKRWYEKSNHKLDSIGSWYQSSATIIIIIVMIVVLLIINAIIIMITIKHLRARNRHPNNKDSEPYVLTNRQ

SEQ ID NO: 77 - protein, 523 aa, Artificial Sequence
  Recombinant parainfluenza virus F sequence
QVDIIKLQRVGILVSKPKSIKISQNFETRYLVLNLIPNIENAQSCGDQQIKQYKKLLDRLIIPLYDGLRLQQDIIVVDNNLKNNTNHRAKRFFGEIIGTIALGVATSAQITAAVALVEAKQARSDIERVKNAVRDTNKAVQSIQGSVGNLIVACKSVQDYVNNEIVPSIKRLGCEAAGLQLGIALTQHYSELTNIFGDNIGTLKEKGIKLQGIASLYHTCITEIFTTSTVDQYDIYDLLFTESIKMRVIDVDLNDYSITLQVRLPLLTKISDAQIYNVDSVSYNIGGTEWYIPLPRNIMTKGAFLGGANLQDCIESFSDYICPSDPGFILNRDIENCLSGNITQCPKTLVISDIVPRYAFVDGGVIANCLSTTCTCNGIDNRINQAPDQGIKIITYKDCQTIGINGMLFKTNQEGTLAAYTPVDITLNNSVNLDPIDLSIELNRARSDLAESKEWYKRSEAKLDSVGSWYQSSTTEIIQIVMIIVLFIINIIVLIVLIKYSRSQNQSMNNHMNEPYILTNKVQ

SEQ ID NO: 78 - protein, 522 aa, Artificial Sequence
  Recombinant parainfluenza virus F sequence
QIDITKLQSVGVLVNSPKGIKISQNFETRYLILSLIPKIEDSHSCGNQQIDQYKKLLDRLIIPLYDGLKLQKDVIVVNHESHNNTNLRTKRFFGEIIGTIAIGIATSAQITAAVALVEAKQARSDIDKLKEAIKDTNKAVQSIQSSVGNLIVACKSVQDYVNNEIVPSITRLGCEAAGLQLGIALTQHYSELTNIFGDNIGTLGEKGVKLQGIASLYRTCITEVFTTSTVDQYDIYDLLFTESIKMRVIDVDLSDYSITLQVRLPLLTKVSNTQIYKVDSISYNIQGKEWYIPLPHHIMTKGAFLGGADIKECIESFSNYICPSDPGFILNHEMENCLSGNITQCPKTIVTSDIVPRYAFVDGGVIANCIPTTCTCNGIDNRINQSPDQGIKIITYKECQIVGINGMLFKTNQEGTLAKYTFDNIKLNNSVALNPIDISLELNKVKSDLEESKRWIEKSNQKLDSIGSWHQSSVTIIIIIVMIVVLLIINAIIIMIMIRYLRDRNRHLNNKDSEPYVLTNRQ

SEQ ID NO: 79 - protein, 522 aa, Artificial Sequence
  Recombinant parainfluenza virus F sequence
QIDITKLQNVGVLVNSPKGIKISQNFETRYLILSLIPKIDDSHSCGNQQIDQYKKLLDRLIIPLYDGLKLQRDVIVVNHESHNNTNLRTKRFFGEIIGTIAIGIATSAQITAAVALVEAKQARSDIDKLKEAIKDTNKAVQSIQSSVGNLIVACKSVQDYVNNEIVPSITRLGCEAAGLQLGIALTQHYSELTNIFGDNIGTLREKGVKLQGIASLYRTCITEVFTTSTVDQYDIYDLLFTESIKMRVIDVDLSDYSITLQVRLPLLTKVSNTQIYKVDSISYNIQGKEWYIPLPHHIMTKGAFLGGADIKECIESFSNYICPSDPGFILNHELENCLSGNITQCPKTIVTSDIVPRYAFVDGGVIANCIPTTCTCNGIDNRINQSPDQGIKIITYKECQIVGINGMLFKTNQEGTLAKYTFDDIKLNNSVALNPIDISLELNKVKSELEESKRWIEKSNHKLDSIGSWYQSSATIIIIIVMIVVLLIINAIIIMITIKHLRARNRHPNNKDSEPYVLTNRQ

SEQ ID NO: 80 - protein, 523 aa, Artificial Sequence
  Recombinant parainfluenza virus F sequence
QVDIIKLQRVGILVSKPKSIKISQNFETRYLVLNLIPNIENAQSCGDQQIKQYKKLLDRLIIPLYDGLRLQQDIIVVDNNLKNNTNHRAKRFFGEIIGTIALGVATSAQITAAVALVEAKQARSDIERVKNAVRDTNKAVQSIQGSVGNLIVACKSVQDYVNNEIVPSIKRLGCEAAGLQLGIALTQHYSELTNIFGDNIGTLKEKGIKLQGIASLYHTCITEIFTTSTVDQYDIYDLLFTESIKMRVIDVDLNDYSITLQVRLPLLTKISDAQIYNVDSVSYNIGGTEWYIPLPRNIMTKGAFLGGANLQDCIESFSDYICPSDPGFILNRDIENCLSGNITQCPKTLVISDIVPRYAFVDGGVIANCLSTTCTCNGIDNRINQAPDQGIKIITYKDCQTIGINGMLFKTNQEGTLAAYTPVDITLNNSVNLDPIDLSIELNRVRSDLAESKEWIKRSEAKLDSVGSWYQSSTTEIIQIVMIIVLFIINIIVLIVLIKYSRSQNQSMNNHMNEPYILTNKVQ

SEQ ID NO: 81 - DNA, 1746 bp, Artificial Sequence
  Recombinant parainfluenza virus F sequence
atgcccatgggcagcctgcagcccctggccaccctgtacctgctgggcatgctggtggcctccgtgctggccggatcccagatccctgtggataagctgagcaacgtgggcgtgatcatcaatgagggcaagctgctgaagatcgccggctcttacgagagccggtatatcgtgctgtccctggtgccatctatcgacctgcaggatggctgcggcaccacacagatcatccagtacaagaacctgctgaatagactgctgatcccactgaaggacgccctggatctgcaggagagcctgatcaccatcacaaatgataccacagtgaccaacgacaatccacagacaaggggctccggagccgtgatcggaaccatcgccctgggagtggcaaccgcagcacagatcacagcaggaatcgccctggccgaggcaagggaggcccgcaaggatatcgccctgatcaaggactctatcgtgaagacccacaatagcgtggagttcatccagcggggcatcggcgagcagatcatcgccctgaagacactgcaggattttgtgaacgacgagatccggcctgccatcggcgagctgagatgtgagacaacagccctgaagctgggcatcaagctgacccagcactactccgagctggccacagccttcagctccaatctgggcaccatcggcgagaagagcctgacactgcaggccctgtctagcctgtattccgccaacatcaccgagatcctgtccacaatcaagaaggacaagtctgatatctacgacatcatctataccgagcaggtgaagggcacagtgatcgacgtggatctggagaagtatatggtgaccctgctggtgaagatcccaatcctgtctgagatcccaggcgtgctgatctacagggcctcctctatcagctataacatcgagggagaggagtggcacgtggcaatccccaactacatcatcaataaggccagctccctgggaggagcagatgtgaccaattgcatcgagtctaagctggcctatatctgtcccagagatcctacacagctgatccctgacaaccagcagaagtgcatcctgggcgacgtgagcaagtgtcccgtgaccaaagtgatcaacaatctggtgcctaagttcgcctttatcaacggcggcgtggtggccaattgcatcgcctccacctgcacatgtggcaccaacagaatccccgtgaatcaggatcgctctaagggcgtgacattcctgacctacacaaactgtggcctgatcggcatcaatggcatcgagctgtatgccaacaagcggggcagagataccacatggggcaatcagatcatcaaggtcggccctgccgtgtccatcaggccagtggacatcagcctgaacctggcctccatcaccaattttctggaggagatcaagacagagctgatgaagatcgaggacaagatcgaggagatcctgtctaaaatctaccacatcgagaacgagatcgcccgcatcaagaagctgatcggcgaggcccccgctagcggaggaggactggaagtgctgttccagggccccgggtctgattacaaggacgatgacgataaaggcagcggctctgcctggtcacatccccagtttgagaagggaggcgggagcggcggagggagcggaggctccgcttggagccatccccagtttgagaaaggcagcgggcaccaccaccaccaccaccaccactga

SEQ ID NO: 82 - DNA, 1770 bp, Artificial Sequence
  Recombinant parainfluenza virus F sequence
atgcccatgggcagcctgcagcccctggccaccctgtacctgctgggcatgctggtggcctccgtgctggccggatccgacgccatcgctggagatcagctgctgaatatcggcgtgattcagtctaagatccggagtctgatgtactataccgacggcggggccagcttcattgtggtcaaactgctgcccaacctgcccccttccaacgggacatgcaatatcacttctctggacgcctacaatgtgaccctgtttaagctgctgacacctctgatcgagaacctgagtaaaatttcaactgtgaccgatacaggaggcgggtcaggaggagggagcggagtggtcgtgggcctggccgctctgggcgtggctactgcagcccagatcaccgctgcagtggcaattgtcaaggcaaacgccaatgccgctgcaatcaacaatctggccagctccattcagagtactaacaaggcagtgtcagacgtgatcgatgccagccggaccattgctacagcagtgcaggctatccaggacagaattaatggcgcaatcgtcaacgggattacatcagccagctgtagggcacacgatgccctgatcggcagcattctgaacctgtacctgactgagctgaccacaatcttccataaccagattacaaatcccgctctgactcctctgtctatccaggcactgcgcattctgctgggcagtaccctgccaatcgtgattgagtcaaagctgaacaccaatttcaacacagccgaactgctgtctagtgggctgctgaccggacagatcatttccatctctcccatgtatatgcagatgctgatccagattaacgtgcccaccttcatcatgcagcccggcgccaaggtcattgacctgatcgctattagcgcaaatcacaaactgcaggaagtcgtggtccaggtgcctaacagaatcctggagtacgccaacgaactgcagaattatcctgctaacgattgcgtggtcacaccaaatagcgtgttttgtcgatacaacgagggctcccctatcccagaatctcagtatcagtgcctgcgggggaatctgaacagctgtactttcaccccaatcattgggaattttctgaagagattcgcctttgctaatggagtgctgtacgctaactgcaaaagcctgctgtgcaggtgtgccgacccaccacacgtggtcagccaggacgatactcagggcatctccatcattgacattaagaggtgttctgagatgatgctggataccttcagttttcgcatcacatcaactttcaacgctacttatgtgaccgacttttccatgatcaatgccaacattgtccatctgagccccctggatctgtccaatcagatcaactctattaataagagcctgaaatccgccgaggactggatcgctgatagtaatttctttgccaaccaggctcgcaccgcaatgaagcagattgaagataagatcgaggaaattctgtctaagatctatcatatcgagaacgaaatcgcacgaattaagaaactgatcggcgaagcccctgctagcggaggaggactggaagtgctgttccagggccccgggtctgattacaaggacgatgacgataaaggcagcggctctgcctggtcacatccccagtttgagaagggaggcgggagcggcggagggagcggaggctccgcttggagccatccccagtttgagaaaggcagcgggcaccaccaccaccaccaccaccactga

SEQ ID NO: 83 - DNA, 1743 bp, Artificial Sequence
  Recombinant parainfluenza virus F sequence
atgcccatgggcagcctgcagcccctggccaccctgtacctgctgggcatgctggtggcctccgtgctggccggatccctggatatcacccacctgatgaacctgggcaccgtgccaacagccatccggtctctggtgtactatacctacacaaagcctagctatctgaccgtggatctgatcccaaacctgaagaatctggaccagaactgcaattacagctccctgaactactataataagacagccctgtccctgatccagcccatcgccgacaacatcaatagactgacaaagcctatcacctccggaggaggctctggaggaggcagcggagccgtgatcggaaccatcgccctgggagtggcaacagcagcacaggtgaccgccgccatcggcctggccaaggcccaggagaacgccaagctgatcctgacactgaagaaggccgccaccgagacaaatgaggccgtgagggatctggccaacagcaataagatcgtggtgaagatgatctccgccatccagaaccagatcaataccatcatccagcctgccatcgatcagatcaattgtcagatcaaggacctgcaggtggccaacatcctgaatctgtatctgaccgagatcaccacagtgttccacaaccagctgacaaatccagccctggagtctatcagcatccaggccctgaagtccctgctgggctctaccctgccagaggtgctgtctaagctggatctgaacaatatcagcgccgcctccgtgatggccagcggactgatcaagggccagatcatcgccgtggacatccctaccatgacactggtgctgatggtgcagatcccatccatctctcccctgcggcaggccaagatcatcgatctgacctctatcacaatccacaccaacagccaggaggtgcaggcagtggtgccagccagagtgctggagatcggctccgagatcctgggcttcgacggcagcgtgtgccagatcacaaaggataccgtgttttgtccatacaatgacgcctatgtgctgcccatccagcagaagcggtgcctgcagggccagaccagagattgcgtgttcaccccagtggcaggcaccttccctcggagatttctgaccacatacggcacaatcgtggccaactgcagggatctggtgtgctcctgtctgcgcccccctcagatcatctatcagcctgacgagaatccagtgaccatcatcgacaaggacctgtgcaccacactgacactggacagcatcaccatcgagatccagaagtctatcaacagcacattcaggcgcgaggtggtgctggagagcacacaggtgaggtccctgaccccactggacctgagcaccgacctgaaccagtttaatcagctgctgaagtccgccgaggaccacatccagagggtgaccgattacctgaactccatcgaggacaagatcgaggagatcctgtctaaaatctaccacatcgagaatgagatcgcccggatcaagaagctgatcggcgaggcccctgctagcggaggaggactggaagtgctgttccagggccccgggtctgattacaaggacgatgacgataaaggcagcggctctgcctggtcacatccccagtttgagaagggaggcgggagcggcggagggagcggaggctccgcttggagccatccccagtttgagaaaggcagcgggcaccaccaccaccaccaccaccactga

SEQ ID NO: 84 - DNA, 1743 bp, Artificial Sequence
  Recombinant parainfluenza virus F sequence
atgcccatgggcagcctgcagcccctggccaccctgtacctgctgggcatgctggtggcctccgtgctggccggatccctggatatcacccacctgatgaacctgggcaccgtgccaacagccatccggtctctggtgtactatacctacacaaagcctagctatctgaccgtggatctgatcccaaacctgaagaatctggaccagaactgcaattacagctccctgaactactataataagacagccctgtccctgatccagcccatcgccgacaacatcaatagactgacaaagcctatcacctccggaggaggctctggaggaggcagcggagccgtgatcggaaccatcgccctgggagtggcaacagcagcacaggtgaccgccgccatcggcctggccaaggcccaggagaacgccaagctgatcctgacactgaagaaggccgccaccgagacaaatgaggccgtgagggatctggccaacagcaataagatcgtggtgaagatgtgctccgccatccagaaccagatcaataccatcatccagcctgccatcgatcagatcaattgtcagatcaaggacctgcaggtggccaacatcctgaatctgtatctgaccgagatcaccacagtgttccacaaccagctgacaaatccagccctggagtctatcagcatccaggccctgaagtccctgctgggctcttgtctgccagaggtgctgtctaagctggatctgaacaatatcagcgccgcctccgtgatggccagcggactgatcaagggccagatcatcgccgtggacatccctaccatgacactggtgctgatggtgcagatcccatccatctctcccctgcggcaggccaagatcatcgatctgacctctatcacaatccacaccaacagccaggaggtgcaggcagtggtgccagccagagtgctggagatcggctccgagatcctgggcttcgacggcagcgtgtgccagatcacaaaggataccgtgttttgtccatacaatgacgcctatgtgctgcccatccagcagaagcggtgcctgcagggccagaccagagattgcgtgttcaccccagtggcaggcaccttccctcggagatttctgaccacatacggcacaatcgtggccaactgcagggatctggtgtgctcctgtctgcgcccccctcagatcatctatcagcctgacgagaatccagtgaccatcatcgacaaggacctgtgcaccacactgacactggacagcatcaccatcgagatccagaagtctatcaacagcacattcaggcgcgaggtggtgctggagagcacacaggtgaggtccctgaccccactggacctgagcaccgacctgaaccagtttaatcagctgctgaagtccgccgaggaccacatccagagggtgaccgattacctgaactccatcgaggacaagatcgaggagatcctgtctaaaatctaccacatcgagaatgagatcgcccggatcaagaagctgatcggcgaggcccctgctagcggaggaggactggaagtgctgttccagggccccgggtctgattacaaggacgatgacgataaaggcagcggctctgcctggtcacatccccagtttgagaagggaggcgggagcggcggagggagcggaggctccgcttggagccatccccagtttgagaaaggcagcgggcaccaccaccaccaccaccaccactga

SEQ ID NO: 85 - DNA, 1644 bp, Artificial Sequence
  Recombinant parainfluenza virus F sequence
ggtaccgccaccatgtactcaatgcagctggcctcttgcgtcacactgacactggtcctgctggtcaactcacagatcgacatcactaaactgcagcacgtcggggtgctggtcaactccccaaagggaatgaaaatttctcagaatttcgagacaagatacctgatcctgagcctgattcccaagatcgaagattcaaacagctgcggggaccagcagattaagcagtacaaacgactgctggatcggctgatcattcctctgtatgatggactgaagctgcagaaagacgtgatcgtcacaaatcaggagtccaacgaaaataccgacccaaggacagagcgcttctttggaggcgtgatcggaactatcgcactgggagtcgctacttctgcacagatcaccgcagctgtggctctggtcgaggccaagcaggctaaaagtgatattgagaagctgaaagaagccatccgagacaccaacaaggctgtgcagagcgtccagagctccgtgggcaatctgattgtcgccatcaagtcagtgcaggattacgtcaacaaagagattgtgcccagcatcgcacgcctggggtgtgaagcagcaggactgcagctgggaatcgcactgacccagcactactccgagctgacaaacatttttggggacaatatcggatctctgcaggaaaagggcatcaagctgcagggcatcgctagtctgtataggacaaatattactgagatcttcaccacatcaactgtggacaagtacgatatctatgacctgctgtttaccgaaagcatcaaggtgagagtgatcgacgtggatctgaacgattattccattactctgcaggtcagactgcctctgctgacaaggctgctgaatactcagatctacaaggtggactccatttcttataacatccagaatcgggagtggtacattccactgccctctcacatcatgaccaagggcgcattcctgggaggcgccgatgtgaaagagtgcattgaagccttctctagttatatctgtcctagcgacccaggatttgtgctgaaccatgagatggaaagttgcctgtcaggcaatattagtcagtgtccacggactaccgtgacctcagatatcgtccccagatacgcatttgtgaacgggggagtggtcgccaattgcatcacaactacctgcacatgtaacgggattggaaacagaatcaatcagccccctgaccagggcgtgaagatcattacacacaaagagtgtaacactatcggcattaatgggatgctgttcaacaccaataaggaaggcacactggccttttatactcctgacgatatcaccctgaacaatagcgtggctctggatccaatcgacatttccatcgagctgaacaaggtgaaatctgacctggaagagagtaaggaatggtatcggagatcaaatcagaaactgagcgctattgaggacaagatcgaggagatcctgagcaagatctaccacatcgagaacgagatcgccagaatcaagaagctgatcggcgaggcccccggaggcctggtgcctcggggcagccaccaccaccaccaccacagtgcttggagccacccacagtttgaaaaatgatgagcggccgcc

SEQ ID NO: 86 - DNA, 1644 bp, Artificial Sequence
  Recombinant parainfluenza virus F sequence
ggtaccgccaccatgtactcaatgcagctggcctcttgcgtcacactgacactggtcctgctggtcaactcacagatcgacatcactaaactgcagcacgtcggggtgctggtcaactccccaaagggaatgaaaatttctcagaatttcgagacaagatacctgatcctgagcctgattcccaagatcgaagattcaaacagctgcggggaccagcagattaagcagtacaaacgactgctggatcggctgatcattcctctgtatgatggactgaagctgcagaaagacgtgatcgtcacaaatcaggagtccaacgaaaataccgacccaaggacagagcgcttctttggaggcgtgatcggaactatcgcactgggagtcgctacttctgcacagatcaccgcagctgtggctctggtcgaggccaagcaggctaaaagtgatattgagaagctgaaagaagccatccgagacaccaacaaggctgtgcagagcgtccagagctccgtgggcaatctgatttgcgccatcaagtcagtgcaggattacgtcaacaaagagattgtgcccagcatcgcacgcctggggtgtgaagcagcaggactgcagctgggaatcgcactgacccagcactactccgagctgacaaacatttttggggacaatatcggatctctgcaggaaaagggcatcaagctgcagggcatcgctagtctgtataggacaaatattactgagtgcttcaccacatcaactgtggacaagtacgatatctatgacctgctgtttaccgaaagcatcaaggtgagagtgatcgacgtggatctgaacgattattccattactctgcaggtcagactgcctctgctgacaaggctgctgaatactcagatctacaaggtggactccatttcttataacatccagaatcgggagtggtacattccactgccctctcacatcatgaccaagggcgcattcctgggaggcgccgatgtgaaagagtgcattgaagccttctctagttatatctgtcctagcgacccaggatttgtgctgaaccatgagatggaaagttgcctgtcaggcaatattagtcagtgtccacggactaccgtgacctcagatatcgtccccagatacgcatttgtgaacgggggagtggtcgccaattgcatcacaactacctgcacatgtaacgggattggaaacagaatcaatcagccccctgaccagggcgtgaagatcattacacacaaagagtgtaacactatcggcattaatgggatgctgttcaacaccaataaggaaggcacactggccttttatactcctgacgatatcaccctgaacaatagcgtggctctggatccaatcgacatttccatcgagctgaacaaggtgaaatctgacctggaagagagtaaggaatggtatcggagatcaaatcagaaactgagcgctattgaggacaagatcgaggagatcctgagcaagatctaccacatcgagaacgagatcgccagaatcaagaagctgatcggcgaggcccccggaggcctggtgcctcggggcagccaccaccaccaccaccacagtgcttggagccacccacagtttgaaaaatgatgagcggccgcc

SEQ ID NO: 87 - DNA, 1644 bp, Artificial Sequence
  Recombinant parainfluenza virus F sequence
ggtaccgccaccatgtactcaatgcagctggcctcttgcgtcacactgacactggtcctgctggtcaactcacagatcgacatcactaaactgcagcacgtcggggtgctggtcaactccccaaagggaatgaaaatttctcagaatttcgagacaagatacctgatcctgagcctgattcccaagatcgaagattcaaacagctgcggggaccagcagattaagcagtacaaacgactgctggatcggctgatcattcctctgtatgatggactgaagctgcagaaagacgtgatcgtcacaaatcaggagtccaacgaaaataccgacccaaggacagagcgcttctttggaggcgtgatcggaactatcgcactgggagtcgctacttctgcacagatcaccgcagctgtggctctggtcgaggccaagcaggctaaaagtgatattgagaagctgaaagaagccatccgagacaccaacaaggctgtgcagagcgtccagagctccgtgggcaatctgattgtcgccatcaagtcagtgcaggattacgtcaacaaagagattgtgcccagcatcgcacgcctggggtgtgaagcagcaggactgcagctgggaatcgcactgacccagcactactccgagctgacaaactgttttggggacaatatcggatctctgcaggaaaagggcatcaagctgcagtgcatcgctagtctgtataggacaaatattactgagatcttcaccacatcaactgtggacaagtacgatatctatgacctgctgtttaccgaaagcatcaaggtgagagtgatcgacgtggatctgaacgattattccattactctgcaggtcagactgcctctgctgacaaggctgctgaatactcagatctacaaggtggactccatttcttataacatccagaatcgggagtggtacattccactgccctctcacatcatgaccaagggcgcattcctgggaggcgccgatgtgaaagagtgcattgaagccttctctagttatatctgtcctagcgacccaggatttgtgctgaaccatgagatggaaagttgcctgtcaggcaatattagtcagtgtccacggactaccgtgacctcagatatcgtccccagatacgcatttgtgaacgggggagtggtcgccaattgcatcacaactacctgcacatgtaacgggattggaaacagaatcaatcagccccctgaccagggcgtgaagatcattacacacaaagagtgtaacactatcggcattaatgggatgctgttcaacaccaataaggaaggcacactggccttttatactcctgacgatatcaccctgaacaatagcgtggctctggatccaatcgacatttccatcgagctgaacaaggtgaaatctgacctggaagagagtaaggaatggtatcggagatcaaatcagaaactgagcgctattgaggacaagatcgaggagatcctgagcaagatctaccacatcgagaacgagatcgccagaatcaagaagctgatcggcgaggcccccggaggcctggtgcctcggggcagccaccaccaccaccaccacagtgcttggagccacccacagtttgaaaaatgatgagcggccgcc

SEQ ID NO: 88 - DNA, 1640 bp, Artificial Sequence
  Recombinant parainfluenza virus F sequence
tctagaccaccatgtactcaatgcagctggcctcttgcgtcacactgacactggtcctgctggtcaactcacagatcgacatcactaaactgcagcacgtcggggtgctggtcaactccccaaagggaatgaaaatttctcagaatttcgagacaagatacctgatcctgagcctgattcccaagatcgaagattcaaacagctgcggggaccagcagattaagcagtacaaacgactgctggatcggctgatcattcctctgtatgattgcctgaagctgcagaaagacgtgatcgtcacaaatcaggagtccaacgaaaataccgacccaaggacagagcgcttctttggaggcgtgatcggaactatcgcactgggagtcgctacttctgcacagatcaccgcagctgtggctctggtcgaggccaagcaggctaaaagtgatattgagaagctgaaagaagccatccgagacaccaacaaggctgtgcagagcgtccagagctccgtgggcaatctgattgtcgccatcaagtcagtgcaggattacgtcaacaaagagattgtgcccagcatcgcacgcctggggtgtgaagcagcaggactgcagctgggaatcgcactgacccagcactactccgagctgacaaacatttttggggacaatatcggatctctgtgcgaaaagggcatcaagctgcagggcatcgctagtctgtataggacaaatattactgagatcttcaccacatcaactgtggacaagtacgatatctatgacctgctgtttaccgaaagcatcaaggtgagagtgatcgacgtggatctgaacgattattccattactctgcaggtcagactgcctctgctgacaaggctgctgaatactcagatctacaaggtggactccatttcttataacatccagaatcgggagtggtacattccactgccctctcacatcatgaccaagggcgcattcctgggaggcgccgatgtgaaagagtgcattgaagccttctctagttatatctgtcctagcgacccaggatttgtgctgaaccatgagatggaaagttgcctgtcaggcaatattagtcagtgtccacggactaccgtgacctcagatatcgtccccagatacgcatttgtgaacgggggagtggtcgccaattgcatcacaactacctgcacatgtaacgggattggaaacagaatcaatcagccccctgaccagggcgtgaagatcattacacacaaagagtgtaacactatcggcattaatgggatgctgttcaacaccaataaggaaggcacactggccttttatactcctgacgatatcaccctgaacaatagcgtggctctggatccaatcgacatttccatcgagctgaacaaggtgaaatctgacctggaagagagtaaggaatggtatcggagatcaaatcagaaactgagcgctattgaggacaagatcgaggagatcctgagcaagatctaccacatcgagaacgagatcgccagaatcaagaagctgatcggcgaggcccccggaggcctggtgcctcggggcagccaccaccaccaccaccacagtgcttggagccacccacagtttgaaaaatgatgaccgcgg

SEQ ID NO: 89 - DNA, 1640 bp, Artificial Sequence
  Recombinant parainfluenza virus F sequence
tctagaccaccatgtactcaatgcagctggcctcttgcgtcacactgacactggtcctgctggtcaactcacagatcgacatcactaaactgcagcacgtcggggtgctggtcaactccccaaagggaatgaaaatttctcagaatttcgagacaagatacctgatcctgagcctgattcccaagatcgaagattcaaacagctgcggggaccagcagattaagcagtacaaacgactgctggatcggctgatcattcctctgtatgatggactgaagctgcagaaagacgtgatcgtcacaaatcaggagtccaacgaaaataccgacccaaggacagagcgcttctttggaggcgtgatcggaactatcgcactgggagtcgctacttctgcacagatcaccgcagctgtggctctggtcgaggccaagcaggctaaaagtgatattgagaagctgaaagaagccatccgagacaccaacaaggctgtgcagagcgtccagagctccgtgggcaatctgattgtcgccatcaagtcagtgcaggattacgtcaacaaagagattgtgcccagcatcgcacgcctggggtgtgaagcagcaggactgcagctgggaatcgcactgacccagcactactccgagctgacaaacatttttgggtgcaatatcggatcttgccaggaaaagggcatcaagctgcagggcatcgctagtctgtataggacaaatattactgagatcttcaccacatcaactgtggacaagtacgatatctatgacctgctgtttaccgaaagcatcaaggtgagagtgatcgacgtggatctgaacgattattccattactctgcaggtcagactgcctctgctgacaaggctgctgaatactcagatctacaaggtggactccatttcttataacatccagaatcgggagtggtacattccactgccctctcacatcatgaccaagggcgcattcctgggaggcgccgatgtgaaagagtgcattgaagccttctctagttatatctgtcctagcgacccaggatttgtgctgaaccatgagatggaaagttgcctgtcaggcaatattagtcagtgtccacggactaccgtgacctcagatatcgtccccagatacgcatttgtgaacgggggagtggtcgccaattgcatcacaactacctgcacatgtaacgggattggaaacagaatcaatcagccccctgaccagggcgtgaagatcattacacacaaagagtgtaacactatcggcattaatgggatgctgttcaacaccaataaggaaggcacactggccttttatactcctgacgatatcaccctgaacaatagcgtggctctggatccaatcgacatttccatcgagctgaacaaggtgaaatctgacctggaagagagtaaggaatggtatcggagatcaaatcagaaactgagcgctattgaggacaagatcgaggagatcctgagcaagatctaccacatcgagaacgagatcgccagaatcaagaagctgatcggcgaggcccccggaggcctggtgcctcggggcagccaccaccaccaccaccacagtgcttggagccacccacagtttgaaaaatgatgaccgcgg

SEQ ID NO: 90 - DNA, 1640 bp, Artificial Sequence
  Recombinant parainfluenza virus F sequence
tctagaccaccatgtactcaatgcagctggcctcttgcgtcacactgacactggtcctgctggtcaactcacagatcgacatcactaaactgcagcacgtcggggtgctggtcaactccccaaagggaatgaaaatttctcagaatttcgagacaagatacctgatcctgagcctgattcccaagatcgaagattcaaacagctgcggggaccagcagattaagcagtacaaacgactgctggatcggctgatcattcctctgtatgatggactgaagctgcagaaagacgtgatcgtcacaaatcaggagtccaacgaaaataccgacccaaggacagagcgcttctttggaggcgtgatcggaactatcgcactgggagtcgctacttctgcacagatcaccgcagctgtggctctggtcgaggccaagcaggctaaaagtgatattgagaagctgaaagaagccatccgagacaccaacaaggctgtgcagagcgtctgcagctccgtgggcaattgcattgtcgccatcaagtcagtgcaggattacgtcaacaaagagattgtgcccagcatcgcacgcctggggtgtgaagcagcaggactgcagctgggaatcgcactgacccagcactactccgagctgacaaacatttttggggacaatatcggatctctgcaggaaaagggcatcaagctgcagggcatcgctagtctgtataggacaaatattactgagatcttcaccacatcaactgtggacaagtacgatatctatgacctgctgtttaccgaaagcatcaaggtgagagtgatcgacgtggatctgaacgattattccattactctgcaggtcagactgcctctgctgacaaggctgctgaatactcagatctacaaggtggactccatttcttataacatccagaatcgggagtggtacattccactgccctctcacatcatgaccaagggcgcattcctgggaggcgccgatgtgaaagagtgcattgaagccttctctagttatatctgtcctagcgacccaggatttgtgctgaaccatgagatggaaagttgcctgtcaggcaatattagtcagtgtccacggactaccgtgacctcagatatcgtccccagatacgcatttgtgaacgggggagtggtcgccaattgcatcacaactacctgcacatgtaacgggattggaaacagaatcaatcagccccctgaccagggcgtgaagatcattacacacaaagagtgtaacactatcggcattaatgggatgctgttcaacaccaataaggaaggcacactggccttttatactcctgacgatatcaccctgaacaatagcgtggctctggatccaatcgacatttccatcgagctgaacaaggtgaaatctgacctggaagagagtaaggaatggtatcggagatcaaatcagaaactgagcgctattgaggacaagatcgaggagatcctgagcaagatctaccacatcgagaacgagatcgccagaatcaagaagctgatcggcgaggcccccggaggcctggtgcctcggggcagccaccaccaccaccaccacagtgcttggagccacccacagtttgaaaaatgatgaccgcgg

SEQ ID NO: 91 - DNA, 1644 bp, Artificial Sequence
  Recombinant parainfluenza virus F sequence
ggtaccgccaccatgtactcaatgcagctggcctcttgcgtcacactgacactggtcctgctggtcaactcacagatcgacatcactaaactgcagcacgtcggggtgctggtcaactccccaaagggaatgaaaatttctcagaatttcgagacaagatacctgatcctgagcctgattcccaagatcgaagattcaaacagctgcggggaccagcagattaagcagtacaaacgactgctggatcggctgatcattcctctgtatgatggactgaagctgcagaaagacgtgatcgtcacaaatcaggagtccaacgaaaataccgacccaaggacagagcgcttctttggaggcgtgatcggaactatcgcactgggagtcgctacttctgcacagatcaccgcagctgtggctctggtcgaggccaagcaggctaaaagtgatattgagaagctgaaagaagccatccgagacaccaacaaggctgtgcagagcgtctgcagctccgtgggcaattgcattgtcgccatcaagtcagtgcaggattacgtcaacaaagagattgtgcccagcatcgcacgcctggggtgtgaagcagcaggactgcagctgggaatcgcactgacccagcactactccgagctgacaaactgttttggggacaatatcggatctctgcaggaaaagggcatcaagctgcagtgcatcgctagtctgtataggacaaatattactgagatcttcaccacatcaactgtggacaagtacgatatctatgacctgctgtttaccgaaagcatcaaggtgagagtgatcgacgtggatctgaacgattattccattactctgcaggtcagactgcctctgctgacaaggctgctgaatactcagatctacaaggtggactccatttcttataacatccagaatcgggagtggtacattccactgccctctcacatcatgaccaagggcgcattcctgggaggcgccgatgtgaaagagtgcattgaagccttctctagttatatctgtcctagcgacccaggatttgtgctgaaccatgagatggaaagttgcctgtcaggcaatattagtcagtgtccacggactaccgtgacctcagatatcgtccccagatacgcatttgtgaacgggggagtggtcgccaattgcatcacaactacctgcacatgtaacgggattggaaacagaatcaatcagccccctgaccagggcgtgaagatcattacacacaaagagtgtaacactatcggcattaatgggatgctgttcaacaccaataaggaaggcacactggccttttatactcctgacgatatcaccctgaacaatagcgtggctctggatccaatcgacatttccatcgagctgaacaaggtgaaatctgacctggaagagagtaaggaatggtatcggagatcaaatcagaaactgagcgctattgaggacaagatcgaggagatcctgagcaagatctaccacatcgagaacgagatcgccagaatcaagaagctgatcggcgaggcccccggaggcctggtgcctcggggcagccaccaccaccaccaccacagtgcttggagccacccacagtttgaaaaatgatgagcggccgcc

SEQ ID NO: 92 - DNA, 1644 bp, Artificial Sequence
  Recombinant parainfluenza virus F sequence
ggtaccgccaccatgtactcaatgcagctggcctcttgcgtcacactgacactggtcctgctggtcaactcacagatcgacatcactaaactgcagcacgtcggggtgctggtcaactccccaaagggaatgaaaatttctcagaatttcgagacaagatacctgatcctgagcctgattcccaagatcgaagattcaaacagctgcggggaccagcagattaagcagtacaaacgactgctggatcggctgatcattcctctgtatgatggactgaagctgcagaaagacgtgatcgtcacaaatcaggagtccaacgaaaataccgacccaaggacagagcgcttctttggaggcgtgatcggaactatcgcactgggagtcgctacttctgcacagatcaccgcagctgtggctctggtcgaggccaagcaggctaaaagtgatattgagaagctgaaagaagccatccgagacaccaacaaggctgtgcagagcgtccagagctccgtgggcaatctgattgtcgcctgcaagtcagtgcaggattacgtcaacaaagagattgtgcccagcatcgcacgcctggggtgtgaagcagcaggactgcagctgggaatcgcactgacccagcactactccgagctgacaaacatttttggggacaatatcggatctctgcaggaaaagggcatcaagctgcagggcatcgctagtctgtataggacatgtattactgagatcttcaccacatcaactgtggacaagtacgatatctatgacctgctgtttaccgaaagcatcaaggtgagagtgatcgacgtggatctgaacgattattccattactctgcaggtcagactgcctctgctgacaaggctgctgaatactcagatctacaaggtggactccatttcttataacatccagaatcgggagtggtacattccactgccctctcacatcatgaccaagggcgcattcctgggaggcgccgatgtgaaagagtgcattgaagccttctctagttatatctgtcctagcgacccaggatttgtgctgaaccatgagatggaaagttgcctgtcaggcaatattagtcagtgtccacggactaccgtgacctcagatatcgtccccagatacgcatttgtgaacgggggagtggtcgccaattgcatcacaactacctgcacatgtaacgggattggaaacagaatcaatcagccccctgaccagggcgtgaagatcattacacacaaagagtgtaacactatcggcattaatgggatgctgttcaacaccaataaggaaggcacactggccttttatactcctgacgatatcaccctgaacaatagcgtggctctggatccaatcgacatttccatcgagctgaacaaggtgaaatctgacctggaagagagtaaggaatggtatcggagatcaaatcagaaactgagcgctattgaggacaagatcgaggagatcctgagcaagatctaccacatcgagaacgagatcgccagaatcaagaagctgatcggcgaggcccccggaggcctggtgcctcggggcagccaccaccaccaccaccacagtgcttggagccacccacagtttgaaaaatgatgagcggccgcc

SEQ ID NO: 93 - protein, 551 aa, parainfluenza virus 5
MGTIIQFLVVSCLLAGTGSIDPAALMQIGVIPTNVRQLMYYTEASSAFIVVKLMPTIDSPISGCNITSISSYNATVTKLLQPIGENLETIRNQLIPTRRRRRFAGVVIGLAALGVATAAQVTAAVALVKANENAAAILNLKNAIQKTNAAVADVVQATQSLGTAVQAVQDHINSVVSPAITAANCKAQDAIIGSILNLYLTELTTIFHNQITNPALSPITIQALRILLGSTLPTVVEKSFNTQISAAELLSSGLLTGQIVGLDLTYMQMVIKVELPTLTVQPATQIIDLATISAFINNQEVMAQLPTRVMVTGSLIQAYPASQCTITPNTVYCRYNDAQVLSDDTMACLQGNLTRCTFSPVVGSFLTRFVLFDGIVYANCRSMLCKCMQPAAVILQPSSSPVTVIDMYKCVSLQLDNLRFTITQLANVTYNSTIKLESSQILPIDPLDISQNLAAVNKSLSDALQHLAQSDTYLSAITSATTTSVLSIIAICLGSLGLILIILLSVVVWKLLTIVAANRNRMEDFVYHNQAFYHSQSDLSEKNRPATLGTR

SEQ ID NO: 94 - protein, 539 aa, human metapneumovirus
MSWKVVIIFSLLITPQHGLKESYLEESCSTITEGYLSVLRTGWYTNVFTLEVGDVENLTCADGPSLIKTELDLTKSALRELRTVSADQLAREEQIENPRQSRFVLGAIALGVATAAAVTAGVAIAKTIRLESEVTAIKNALKKTNEAVSTLGNGVRVLATAVRELKDFVSKNLTRAINKNKCDIADLKMAVSFSQFNRRFLNVVRQFSDNAGITPAISLDLMTDAELARAVSNMPTSAGQIKLMLENRAMVRRKGFGFLIGVYGSSVIYMVQLPIFGVIDTPCWIVKAAPSCSGKKGNYACLLREDQGWYCQNAGSTVYYPNEKDCETRGDHVFCDTAAGINVAEQSKECNINISTTNYPCKVSTGRHPISMVALSPLGALVACYKGVSCSIGSNRVGIIKQLNKGCSYITNQDADTVTIDNTVYQLSKVEGEQHVIKGRPVSSSFDPVKFPEDQFNVALDQVFESIENSQALVDQSNRILSSAEKGNTGFIIVIILIAVLGSTMILVSVFIIIKKTKKPTGAPPELSGVTNNGFIPHN

SEQ ID NO: 95 - protein, 574 aa, Human respiratory syncytial virus
MELLIHRLSAIFLTLAINALYLTSSQNITEEFYQSTCSAVSRGYFSALRTGWYTSVITIELSNIKETKCNGTDTKVKLIKQELDKYKNAVTELQLLMQNTPAANNRARREAPQYMNYTINTTKNLNVSISKKRKRRFLGFLLGVGSAIASGIAVSKVLHLEGEVNKIKNALLSTNKAVVSLSNGVSVLTSKVLDLKNYINNQLLPIVNQQSCRISNIETVIEFQQKNSRLLEINREFSVNAGVTTPLSTYMLTNSELLSLINDMPITNDQKKLMSSNVQIVRQQSYSIMSIIKEEVLAYVVQLPIYGVIDTPCWKLHTSPLCTTNIKEGSNICLTRTDRGWYCDNAGSVSFFPQADTCKVQSNRVFCDTMNSLTLPSEVSLCNTDIFNSKYDCKIMTSKTDISSSVITSLGAIVSCYGKTKCTASNKNRGIIKTFSNGCDYVSNKGVDTVSVGNTLYYVNKLEGKNLYVKGEPIINYYDPLVFPSDEFDASISQVNEKINQSLAFIRRSDELLHNVNTGKSTTNIMITTIIIVIIVVLLSLIAIGLLLYCKAKNTPVTLSKDQLSGINNIAFSK